European Patent Application EP 4 549 449 A2, published May 7, 2025. Title: RNA CONSTRUCTS AND USES THEREOF. Applicant: BioNTech SE. Application EP. The sequence listing filed with the application follows.

SEQUENCE LISTING (41 sequences)

SEQ ID NO: 1-7 - skipped (7 entries)

SEQ ID NO: 8 - RNA, 20 nt, synthetic construct
  source 1..20: mol_type = other RNA
gagtcgctagccgcgtcgct

SEQ ID NO: 9 - protein, 1273 aa, synthetic construct
MFVFLVLLPLVSSQCVNLTTRTQLPPAYTNSFTRGVYYPDKVFRSSVLHSTQDLFLPFFSNVTWFHAIHVSGTNGTKRFDNPVLPFNDGVYFASTEKSNIIRGWIFGTTLDSKTQSLLIVNNATNVVIKVCEFQFCNDPFLGVYYHKNNKSWMESEFRVYSSANNCTFEYVSQPFLMDLEGKQGNFKNLREFVFKNIDGYFKIYSKHTPINLVRDLPQGFSALEPLVDLPIGINITRFQTLLALHRSYLTPGDSSSGWTAGAAAYYVGYLQPRTFLLKYNENGTITDAVDCALDPLSETKCTLKSFTVEKGIYQTSNFRVQPTESIVRFPNITNLCPFGEVFNATRFASVYAWNRKRISNCVADYSVLYNSASFSTFKCYGVSPTKLNDLCFTNVYADSFVIRGDEVRQIAPGQTGKIADYNYKLPDDFTGCVIAWNSNNLDSKVGGNYNYLYRLFRKSNLKPFERDISTEIYQAGSTPCNGVEGFNCYFPLQSYGFQPTNGVGYQPYRVVVLSFELLHAPATVCGPKKSTNLVKNKCVNFNFNGLTGTGVLTESNKKFLPFQQFGRDIADTTDAVRDPQTLEILDITPCSFGGVSVITPGTNTSNQVAVLYQDVNCTEVPVAIHADQLTPTWRVYSTGSNVFQTRAGCLIGAEHVNNSYECDIPIGAGICASYQTQTNSPRRARSVASQSIIAYTMSLGAENSVAYSNNSIAIPTNFTISVTTEILPVSMTKTSVDCTMYICGDSTECSNLLLQYGSFCTQLNRALTGIAVEQDKNTQEVFAQVKQIYKTPPIKDFGGFNFSQILPDPSKPSKRSFIEDLLFNKVTLADAGFIKQYGDCLGDIAARDLICAQKFNGLTVLPPLLTDEMIAQYTSALLAGTITSGWTFGAGAALQIPFAMQMAYRFNGIGVTQNVLYENQKLIANQFNSAIGKIQDSLSSTASALGKLQDVVNQNAQALNTLVKQLSSNFGAISSVLNDILSRLDPPEAEVQIDRLITGRLQSLQTYVTQQLIRAAEIRASANLAATKMSECVLGQSKRVDFCGKGYHLMSFPQSAPHGVVFLHVTYVPAQEKNFTTAPAICHDGKAHFPREGVFVSNGTHWFVTQRNFYEPQIITTDNTFVSGNCDVVIGIVNNTVYDPLQPELDSFKEELDKYFKNHTSPDVDLGDISGINASVVNIQKEIDRLNEVAKNLNESLIDLQELGKYEQYIKWPWYIWLGFIAGLIAIVMVTIMLCCMTSCCSCLKGCCSCGSCCKFDEDDSEPVLKGVKLHYT

SEQ ID NO: 10 - RNA, 4283 nt, synthetic construct
  source 1..4283: mol_type = other RNA
agaataaactagtattcttctggtccccacagactcagagagaacccgccaccatgttcgtgttcctggtgctgctgcctctggtgtccagccagtgtgtgaacctgaccaccagaacacagctgcctccagcctacaccaacagctttaccagaggcgtgtactaccccgacaaggtgttcagatccagcgtgctgcactctacccaggacctgttcctgcctttcttcagcaacgtgacctggttccacgccatccacgtgtccggcaccaatggcaccaagagattcgacaaccccgtgctgcccttcaacgacggggtgtactttgccagcaccgagaagtccaacatcatcagaggctggatcttcggcaccacactggacagcaagacccagagcctgctgatcgtgaacaacgccaccaacgtggtcatcaaagtgtgcgagttccagttctgcaacgaccccttcctgggcgtctactaccacaagaacaacaagagctggatggaaagcgagttccgggtgtacagcagcgccaacaactgcaccttcgagtacgtgtcccagcctttcctgatggacctggaaggcaagcagggcaacttcaagaacctgcgcgagttcgtgtttaagaacatcgacggctacttcaagatctacagcaagcacacccctatcaacctcgtgcgggatctgcctcagggcttctctgctctggaacccctggtggatctgcccatcggcatcaacatcacccggtttcagacactgctggccctgcacagaagctacctgacacctggcgatagcagcagcggatggacagctggtgccgccgcttactatgtgggctacctgcagcctagaaccttcctgctgaagtacaacgagaacggcaccatcaccgacgccgtggattgtgctctggatcctctgagcgagacaaagtgcaccctgaagtccttcaccgtggaaaagggcatctaccagaccagcaacttccgggtgcagcccaccgaatccatcgtgcggttccccaatatcaccaatctgtgccccttcggcgaggtgttcaatgccaccagattcgcctctgtgtacgcctggaaccggaagcggatcagcaattgcgtggccgactactccgtgctgtacaactccgccagcttcagcaccttcaagtgctacggcgtgtcccctaccaagctgaacgacctgtgcttcacaaacgtgtacgccgacagcttcgtgatccggggagatgaagtgcggcagattgcccctggacagacaggcaagatcgccgactacaactacaagctgcccgacgacttcaccggctgtgtgattgcctggaacagcaacaacctggactccaaagtcggcggcaactacaattacctgtaccggctgttccggaagtccaatctgaagcccttcgagcgggacatctccaccgagatctatcaggccggcagcaccccttgtaacggcgtggaaggcttcaactgctacttcccactgcagtcctacggctttcagcccacaaatggcgtgggctatcagccctacagagtggtggtgctgagcttcgaactgctgcatgcccctgccacagtgtgcggccctaagaaaagcaccaatctcgtgaagaacaaatgcgtgaacttcaacttcaacggcctgaccggcaccggcgtgctgacagagagcaacaagaagttcctgccattccagcagtttggccgggatatcgccgataccacagacgccgttagagatccccagacactggaaatcctggacatcaccccttgcagcttcggcggagtgtctgtgatcacccctggcaccaacaccagcaatcaggtggcagtgctgtaccaggacgtgaactgtaccgaagtgcccgtggccattcacgccgatcagctgacacctacatggcgggtgtactccaccggcagcaatgtgtttcagaccagagccggctgtctgatcggagccgagcacgtgaacaatagctacgagtgcgacatccccatcggcgctggaatctgcgccagctaccagacacagacaaacagccctcggagagccagaagcgtggccagccagagcatcattgcctacacaatgtctctgggcgccgagaacagcgtggcctactccaacaactctatcgctatccccaccaacttcaccatcagcgtgaccacagagatcctgcctgtgtccatgaccaagaccagcgtggactgcaccatgtacatctgcggcgattccaccgagtgctccaacctgctgctgcagtacggcagcttctgcacccagctgaatagagccctgacagggatcgccgtggaacaggacaagaacacccaagaggtgttcgcccaagtgaagcagatctacaagacccctcctatcaaggacttcggcggcttcaatttcagccagattctgcccgatcctagcaagcccagcaagcggagcttcatcgaggacctgctgttcaacaaagtgacactggccgacgccggcttcatcaagcagtatggcgattgtctgggcgacattgccgccagggatctgatttgcgcccagaagtttaacggactgacagtgctgcctcctctgctgaccgatgagatgatcgcccagtacacatctgccctgctggccggcacaatcacaagcggctggacatttggagcaggcgccgctctgcagatcccctttgctatgcagatggcctaccggttcaacggcatcggagtgacccagaatgtgctgtacgagaaccagaagctgatcgccaaccagttcaacagcgccatcggcaagatccaggacagcctgagcagcacagcaagcgccctgggaaagctgcaggacgtggtcaaccagaatgcccaggcactgaacaccctggtcaagcagctgtcctccaacttcggcgccatcagctctgtgctgaacgatatcctgagcagactggaccctcctgaggccgaggtgcagatcgacagactgatcacaggcagactgcagagcctccagacatacgtgacccagcagctgatcagagccgccgagattagagcctctgccaatctggccgccaccaagatgtctgagtgtgtgctgggccagagcaagagagtggacttttgcggcaagggctaccacctgatgagcttccctcagtctgcccctcacggcgtggtgtttctgcacgtgacatatgtgcccgctcaagagaagaatttcaccaccgctccagccatctgccacgacggcaaagcccactttcctagagaaggcgtgttcgtgtccaacggcacccattggttcgtgacacagcggaacttctacgagccccagatcatcaccaccgacaacaccttcgtgtctggcaactgcgacgtcgtgatcggcattgtgaacaataccgtgtacgaccctctgcagcccgagctggacagcttcaaagaggaactggacaagtactttaagaaccacacaagccccgacgtggacctgggcgatatcagcggaatcaatgccagcgtcgtgaacatccagaaagagatcgaccggctgaacgaggtggccaagaatctgaacgagagcctgatcgacctgcaagaactggggaagtacgagcagtacatcaagtggccctggtacatctggctgggctttatcgccggactgattgccatcgtgatggtcacaatcatgctgtgttgcatgaccagctgctgtagctgcctgaagggctgttgtagctgtggcagctgctgcaagttcgacgaggacgattctgagcccgtgctgaagggcgtgaaactgcactacacatgatgactcgagctggtactgcatgcacgcaatgctagctgcccctttcccgtcctgggtaccccgagtctcccccgacctcgggtcccaggtatgctcccacctccacctgccccactcaccacctctgctagttccagacacctcccaagcacgcagcaatgcagctcaaaacgcttagcctagccacacccccacgggaaacagcagtgattaacctttagcaataaacgaaagtttaactaagctatactaaccccagggttggtcaatttcgtgccagccacaccctggagctagcaaaaaaaaaaaaaaaaaaaaaaaaaaaaaagcatatgactaaaaaaaaaaaaaaaaaaaaaaaaaaaaaaaaaaaaaaaaaaaaaaaaaaaaaaaaaaaaaaaaaaaaaa

SEQ ID NO: 11 - RNA, 47 nt, synthetic construct
  source 1..47: mol_type = other RNA
agaataaactagtattcttctggtccccacagactcagagagaaccc

SEQ ID NO: 12 - RNA, 42 nt, synthetic construct
  source 1..42: mol_type = other RNA
aaactagtattcttctggtccccacagactcagagagaaccc

SEQ ID NO: 13 - RNA, 278 nt, synthetic construct
  source 1..278: mol_type = other RNA
ctggtactgcatgcacgcaatgctagctgcccctttcccgtcctgggtaccccgagtctcccccgacctcgggtcccaggtatgctcccacctccacctgccccactcaccacctctgctagttccagacacctcccaagcacgcagcaatgcagctcaaaacgcttagcctagccacacccccacgggaaacagcagtgattaacctttagcaataaacgaaagtttaactaagctatactaaccccagggttggtcaatttcgtgccagccacacc

SEQ ID NO: 14 - RNA, 110 nt, synthetic construct
  source 1..110: mol_type = other RNA
aaaaaaaaaaaaaaaaaaaaaaaaaaaaaagcatatgactaaaaaaaaaaaaaaaaaaaaaaaaaaaaaaaaaaaaaaaaaaaaaaaaaaaaaaaaaaaaaaaaaaaaaa

SEQ ID NO: 15 - RNA, 458 nt, synthetic construct
  source 1..458: mol_type = other RNA
agaataaactagtattcttctggtccccacagactcagagagaacccgccaccctcgagctggtactgcatgcacgcaatgctagctgcccctttcccgtcctgggtaccccgagtctcccccgacctcgggtcccaggtatgctcccacctccacctgccccactcaccacctctgctagttccagacacctcccaagcacgcagcaatgcagctcaaaacgcttagcctagccacacccccacgggaaacagcagtgattaacctttagcaataaacgaaagtttaactaagctatactaaccccagggttggtcaatttcgtgccagccacaccctggagctagcaaaaaaaaaaaaaaaaaaaaaaaaaaaaaagcatatgactaaaaaaaaaaaaaaaaaaaaaaaaaaaaaaaaaaaaaaaaaaaaaaaaaaaaaaaaaaaaaaaaaaaaaa

SEQ ID NO: 16 - RNA, 4283 nt, synthetic construct; identical to SEQ ID NO: 10
  source 1..4283: mol_type = other RNA

SEQ ID NO: 17 - protein, 1273 aa, synthetic construct
  REGION 1..1273: note = S protein
MFVFLVLLPLVSSQCVNLTTRTQLPPAYTNSFTRGVYYPDKVFRSSVLHSTQDLFLPFFSNVTWFHAIHVSGTNGTKRFDNPVLPFNDGVYFASTEKSNIIRGWIFGTTLDSKTQSLLIVNNATNVVIKVCEFQFCNDPFLGVYYHKNNKSWMESEFRVYSSANNCTFEYVSQPFLMDLEGKQGNFKNLREFVFKNIDGYFKIYSKHTPINLVRDLPQGFSALEPLVDLPIGINITRFQTLLALHRSYLTPGDSSSGWTAGAAAYYVGYLQPRTFLLKYNENGTITDAVDCALDPLSETKCTLKSFTVEKGIYQTSNFRVQPTESIVRFPNITNLCPFGEVFNATRFASVYAWNRKRISNCVADYSVLYNSASFSTFKCYGVSPTKLNDLCFTNVYADSFVIRGDEVRQIAPGQTGKIADYNYKLPDDFTGCVIAWNSNNLDSKVGGNYNYLYRLFRKSNLKPFERDISTEIYQAGSTPCNGVEGFNCYFPLQSYGFQPTNGVGYQPYRVVVLSFELLHAPATVCGPKKSTNLVKNKCVNFNFNGLTGTGVLTESNKKFLPFQQFGRDIADTTDAVRDPQTLEILDITPCSFGGVSVITPGTNTSNQVAVLYQDVNCTEVPVAIHADQLTPTWRVYSTGSNVFQTRAGCLIGAEHVNNSYECDIPIGAGICASYQTQTNSPRRARSVASQSIIAYTMSLGAENSVAYSNNSIAIPTNFTISVTTEILPVSMTKTSVDCTMYICGDSTECSNLLLQYGSFCTQLNRALTGIAVEQDKNTQEVFAQVKQIYKTPPIKDFGGFNFSQILPDPSKPSKRSFIEDLLFNKVTLADAGFIKQYGDCLGDIAARDLICAQKFNGLTVLPPLLTDEMIAQYTSALLAGTITSGWTFGAGAALQIPFAMQMAYRFNGIGVTQNVLYENQKLIANQFNSAIGKIQDSLSSTASALGKLQDVVNQNAQALNTLVKQLSSNFGAISSVLNDILSRLDKVEAEVQIDRLITGRLQSLQTYVTQQLIRAAEIRASANLAATKMSECVLGQSKRVDFCGKGYHLMSFPQSAPHGVVFLHVTYVPAQEKNFTTAPAICHDGKAHFPREGVFVSNGTHWFVTQRNFYEPQIITTDNTFVSGNCDVVIGIVNNTVYDPLQPELDSFKEELDKYFKNHTSPDVDLGDISGINASVVNIQKEIDRLNEVAKNLNESLIDLQELGKYEQYIKWPWYIWLGFIAGLIAIVMVTIMLCCMTSCCSCLKGCCSCGSCCKFDEDDSEPVLKGVKLHYT

SEQ ID NO: 18 - RNA, 3819 nt, synthetic construct
  source 1..3819: mol_type = other RNA
atgtttgtgtttcttgtgctgctgcctcttgtgtcttctcagtgtgtgaatttgacaacaagaacacagctgccaccagcttatacaaattcttttaccagaggagtgtattatcctgataaagtgtttagatcttctgtgctgcacagcacacaggacctgtttctgccattttttagcaatgtgacatggtttcatgcaattcatgtgtctggaacaaatggaacaaaaagatttgataatcctgtgctgccttttaatgatggagtgtattttgcttcaacagaaaagtcaaatattattagaggatggatttttggaacaacactggattctaaaacacagtctctgctgattgtgaataatgcaacaaatgtggtgattaaagtgtgtgaatttcagttttgtaatgatccttttctgggagtgtattatcacaaaaataataaatcttggatggaatctgaatttagagtgtattcctctgcaaataattgtacatttgaatatgtgtctcagccttttctgatggatctggaaggaaaacagggcaattttaaaaatctgagagaatttgtgtttaaaaatattgatggatattttaaaatttattctaaacacacaccaattaatttagtgagagatctgcctcagggattttctgctctggaacctctggtggatctgccaattggcattaatattacaagatttcagacactgctggctctgcacagatcttatctgacacctggagattcttcttctggatggacagccggagctgcagcttattatgtgggctatctgcagccaagaacatttctgctgaaatataatgaaaatggaacaattacagatgctgtggattgtgctctggatcctctgtctgaaacaaaatgtacattaaaatcttttacagtggaaaaaggcatttatcagacatctaattttagagtgcagccaacagaatctattgtgagatttccaaatattacaaatctgtgtccatttggagaagtgtttaatgcaacaagatttgcatctgtgtatgcatggaatagaaaaagaatttctaattgtgtggctgattattctgtgctgtataatagtgcttctttttccacatttaaatgttatggagtgtctccaacaaaattaaatgatttatgttttacaaatgtgtatgctgattcttttgtgatcagaggtgatgaagtgagacagattgcccccggacagacaggaaaaattgctgattacaattacaaactgcctgatgattttacaggatgtgtgattgcttggaattctaataatttagattctaaagtgggaggaaattacaattatctgtacagactgtttagaaaatcaaatctgaaaccttttgaaagagatatttcaacagaaatttatcaggctggatcaacaccttgtaatggagtggaaggatttaattgttattttccattacagagctatggatttcagccaaccaatggtgtgggatatcagccatatagagtggtggtgctgtcttttgaactgctgcatgcacctgcaacagtgtgtggacctaaaaaatctacaaatttagtgaaaaataaatgtgtgaattttaattttaatggattaacaggaacaggagtgctgacagaatctaataaaaaatttctgccttttcagcagtttggcagagatattgcagataccacagatgcagtgagagatcctcagacattagaaattctggatattacaccttgttcttttgggggtgtgtctgtgattacacctggaacaaatacatctaatcaggtggctgtgctgtatcaggatgtgaattgtacagaagtgccagtggcaattcatgcagatcagctgacaccaacatggagagtgtattctacaggatctaatgtgtttcagacaagagcaggatgtctgattggagcagaacatgtgaataattcttatgaatgtgatattccaattggagcaggcatttgtgcatcttatcagacacagacaaattccccaaggagagcaagatctgtggcatctcagtctattattgcatacaccatgtctctgggagcagaaaattctgtggcatattctaataattctattgctattccaacaaattttaccatttctgtgacaacagaaattttacctgtgtctatgacaaaaacatctgtggattgtaccatgtacatttgtggagattctacagaatgttctaatctgctgctgcagtatggatctttttgtacacagctgaatagagctttaacaggaattgctgtggaacaggataaaaatacacaggaagtgtttgctcaggtgaaacagatttacaaaacaccaccaattaaagattttggaggatttaattttagccagattctgcctgatccttctaaaccttctaaaagatcttttattgaagatctgctgtttaataaagtgacactggcagatgcaggatttattaaacagtatggagattgcctgggtgatattgctgcaagagatctgatttgtgctcagaaatttaatggactgacagtgctgcctcctctgctgacagatgaaatgattgctcagtacacatctgctttactggctggaacaattacaagcggatggacatttggagctggagctgctctgcagattccttttgcaatgcagatggcttacagatttaatggaattggagtgacacagaatgtgttatatgaaaatcagaaactgattgcaaatcagtttaattctgcaattggcaaaattcaggattctctgtcttctacagcttctgctctgggaaaactgcaggatgtggtgaatcagaatgcacaggcactgaatactctggtgaaacagctgtctagcaattttggggcaatttcttctgtgctgaatgatattctgtctagactggataaagtggaagctgaagtgcagattgatagactgatcacaggaagactgcagtctctgcagacttatgtgacacagcagctgattagagctgctgaaattagagcttctgctaatctggctgctacaaaaatgtctgaatgtgtgctgggacagtcaaaaagagtggatttttgtggaaaaggatatcatctgatgtcttttccacagtctgctccacatggagtggtgtttttacatgtgacatatgtgccagcacaggaaaagaattttaccacagcaccagcaatttgtcatgatggaaaagcacattttccaagagaaggagtgtttgtgtctaatggaacacattggtttgtgacacagagaaatttttatgaacctcagattattacaacagataatacatttgtgtcaggaaattgtgatgtggtgattggaattgtgaataatacagtgtatgatccactgcagccagaactggattcttttaaagaagaactggataaatattttaaaaatcacacatctcctgatgtggatttaggagatatttctggaatcaatgcatctgtggtgaatattcagaaagaaattgatagactgaatgaagtggccaaaaatctgaatgaatctctgattgatctgcaggaacttggaaaatatgaacagtacattaaatggccttggtacatttggcttggatttattgcaggattaattgcaattgtgatggtgacaattatgttatgttgtatgacatcatgttgttcttgtttaaaaggatgttgttcttgtggaagctgttgtaaatttgatgaagatgattctgaacctgtgttaaaaggagtgaaattgcattacaca

SEQ ID NO: 19 - protein, 218 aa, synthetic construct
MFVFLVLLPLVSSQCVVRFPNITNLCPFGEVFNATRFASVYAWNRKRISNCVADYSVLYNSASFSTFKCYGVSPTKLNDLCFTNVYADSFVIRGDEVRQIAPGQTGKIADYNYKLPDDFTGCVIAWNSNNLDSKVGGNYNYLYRLFRKSNLKPFERDISTEIYQAGSTPCNGVEGFNCYFPLQSYGFQPTNGVGYQPYRVVVLSFELLHAPATVCGPK

SEQ ID NO: 20 - RNA, 654 nt, synthetic construct
  source 1..654: mol_type = other RNA
atgtttgtgtttcttgtgctgctgcctcttgtgtcttctcagtgtgtggtgagatttccaaatattacaaatctgtgtccatttggagaagtgtttaatgcaacaagatttgcatctgtgtatgcatggaatagaaaaagaatttctaattgtgtggctgattattctgtgctgtataatagtgcttctttttccacatttaaatgttatggagtgtctccaacaaaattaaatgatttatgttttacaaatgtgtatgctgattcttttgtgatcagaggtgatgaagtgagacagattgcccccggacagacaggaaaaattgctgattacaattacaaactgcctgatgattttacaggatgtgtgattgcttggaattctaataatttagattctaaagtgggaggaaattacaattatctgtacagactgtttagaaaatcaaatctgaaaccttttgaaagagatatttcaacagaaatttatcaggctggatcaacaccttgtaatggagtggaaggatttaattgttattttccattacagagctatggatttcagccaaccaatggtgtgggatatcagccatatagagtggtggtgctgtcttttgaactgctgcatgcacctgcaacagtgtgtggacctaaa

SEQ ID NO: 21 - protein, 266 aa, synthetic construct
MFVFLVLLPLVSSQCVVRFPNITNLCPFGEVFNATRFASVYAWNRKRISNCVADYSVLYNSASFSTFKCYGVSPTKLNDLCFTNVYADSFVIRGDEVRQIAPGQTGKIADYNYKLPDDFTGCVIAWNSNNLDSKVGGNYNYLYRLFRKSNLKPFERDISTEIYQAGSTPCNGVEGFNCYFPLQSYGFQPTNGVGYQPYRVVVLSFELLHAPATVCGPKGSPGSGSGSGYIPEAPRDGQAYVRKDGEWVLLSTFLGRSLEVLFQGPG

SEQ ID NO: 22 - RNA, 798 nt, synthetic construct
  source 1..798: mol_type = other RNA
atgtttgtgtttcttgtgctgctgcctcttgtgtcttctcagtgtgtggtgagatttccaaatattacaaatctgtgtccatttggagaagtgtttaatgcaacaagatttgcatctgtgtatgcatggaatagaaaaagaatttctaattgtgtggctgattattctgtgctgtataatagtgcttctttttccacatttaaatgttatggagtgtctccaacaaaattaaatgatttatgttttacaaatgtgtatgctgattcttttgtgatcagaggtgatgaagtgagacagattgcccccggacagacaggaaaaattgctgattacaattacaaactgcctgatgattttacaggatgtgtgattgcttggaattctaataatttagattctaaagtgggaggaaattacaattatctgtacagactgtttagaaaatcaaatctgaaaccttttgaaagagatatttcaacagaaatttatcaggctggatcaacaccttgtaatggagtggaaggatttaattgttattttccattacagagctatggatttcagccaaccaatggtgtgggatatcagccatatagagtggtggtgctgtcttttgaactgctgcatgcacctgcaacagtgtgtggacctaaaggctcccccggctccggctccggatctggttatattcctgaagctccaagagatgggcaagcttacgttcgtaaagatggcgaatgggtattactttctacctttttaggccggtccctggaggtgctgttccagggccccggc

SEQ ID NO: 23 - RNA, 3819 nt, synthetic construct
  source 1..3819: mol_type = other RNA
atgtttgtgtttcttgtgctgctgcctcttgtgtcttctcagtgtgtgaatttgacaacaagaacacagctgccaccagcttatacaaattcttttaccagaggagtgtattatcctgataaagtgtttagatcttctgtgctgcacagcacacaggacctgtttctgccattttttagcaatgtgacatggtttcatgcaattcatgtgtctggaacaaatggaacaaaaagatttgataatcctgtgctgccttttaatgatggagtgtattttgcttcaacagaaaagtcaaatattattagaggatggatttttggaacaacactggattctaaaacacagtctctgctgattgtgaataatgcaacaaatgtggtgattaaagtgtgtgaatttcagttttgtaatgatccttttctgggagtgtattatcacaaaaataataaatcttggatggaatctgaatttagagtgtattcctctgcaaataattgtacatttgaatatgtgtctcagccttttctgatggatctggaaggaaaacagggcaattttaaaaatctgagagaatttgtgtttaaaaatattgatggatattttaaaatttattctaaacacacaccaattaatttagtgagagatctgcctcagggattttctgctctggaacctctggtggatctgccaattggcattaatattacaagatttcagacactgctggctctgcacagatcttatctgacacctggagattcttcttctggatggacagccggagctgcagcttattatgtgggctatctgcagccaagaacatttctgctgaaatataatgaaaatggaacaattacagatgctgtggattgtgctctggatcctctgtctgaaacaaaatgtacattaaaatcttttacagtggaaaaaggcatttatcagacatctaattttagagtgcagccaacagaatctattgtgagatttccaaatattacaaatctgtgtccatttggagaagtgtttaatgcaacaagatttgcatctgtgtatgcatggaatagaaaaagaatttctaattgtgtggctgattattctgtgctgtataatagtgcttctttttccacatttaaatgttatggagtgtctccaacaaaattaaatgatttatgttttacaaatgtgtatgctgattcttttgtgatcagaggtgatgaagtgagacagattgcccccggacagacaggaaaaattgctgattacaattacaaactgcctgatgattttacaggatgtgtgattgcttggaattctaataatttagattctaaagtgggaggaaattacaattatctgtacagactgtttagaaaatcaaatctgaaaccttttgaaagagatatttcaacagaaatttatcaggctggatcaacaccttgtaatggagtggaaggatttaattgttattttccattacagagctatggatttcagccaaccaatggtgtgggatatcagccatatagagtggtggtgctgtcttttgaactgctgcatgcacctgcaacagtgtgtggacctaaaaaatctacaaatttagtgaaaaataaatgtgtgaattttaattttaatggattaacaggaacaggagtgctgacagaatctaataaaaaatttctgccttttcagcagtttggcagagatattgcagataccacagatgcagtgagagatcctcagacattagaaattctggatattacaccttgttcttttgggggtgtgtctgtgattacacctggaacaaatacatctaatcaggtggctgtgctgtatcaggatgtgaattgtacagaagtgccagtggcaattcatgcagatcagctgacaccaacatggagagtgtattctacaggatctaatgtgtttcagacaagagcaggatgtctgattggagcagaacatgtgaataattcttatgaatgtgatattccaattggagcaggcatttgtgcatcttatcagacacagacaaattccccaaggagagcaagatctgtggcatctcagtctattattgcatacaccatgtctctgggagcagaaaattctgtggcatattctaataattctattgctattccaacaaattttaccatttctgtgacaacagaaattttacctgtgtctatgacaaaaacatctgtggattgtaccatgtacatttgtggagattctacagaatgttctaatctgctgctgcagtatggatctttttgtacacagctgaatagagctttaacaggaattgctgtggaacaggataaaaatacacaggaagtgtttgctcaggtgaaacagatttacaaaacaccaccaattaaagattttggaggatttaattttagccagattctgcctgatccttctaaaccttctaaaagatcttttattgaagatctgctgtttaataaagtgacactggcagatgcaggatttattaaacagtatggagattgcctgggtgatattgctgcaagagatctgatttgtgctcagaaatttaatggactgacagtgctgcctcctctgctgacagatgaaatgattgctcagtacacatctgctttactggctggaacaattacaagcggatggacatttggagctggagctgctctgcagattccttttgcaatgcagatggcttacagatttaatggaattggagtgacacagaatgtgttatatgaaaatcagaaactgattgcaaatcagtttaattctgcaattggcaaaattcaggattctctgtcttctacagcttctgctctgggaaaactgcaggatgtggtgaatcagaatgcacaggcactgaatactctggtgaaacagctgtctagcaattttggggcaatttcttctgtgctgaatgatattctgtctagactggatcctcctgaagctgaagtgcagattgatagactgatcacaggaagactgcagtctctgcagacttatgtgacacagcagctgattagagctgctgaaattagagcttctgctaatctggctgctacaaaaatgtctgaatgtgtgctgggacagtcaaaaagagtggatttttgtggaaaaggatatcatctgatgtcttttccacagtctgctccacatggagtggtgtttttacatgtgacatatgtgccagcacaggaaaagaattttaccacagcaccagcaatttgtcatgatggaaaagcacattttccaagagaaggagtgtttgtgtctaatggaacacattggtttgtgacacagagaaatttttatgaacctcagattattacaacagataatacatttgtgtcaggaaattgtgatgtggtgattggaattgtgaataatacagtgtatgatccactgcagccagaactggattcttttaaagaagaactggataaatattttaaaaatcacacatctcctgatgtggatttaggagatatttctggaatcaatgcatctgtggtgaatattcagaaagaaattgatagactgaatgaagtggccaaaaatctgaatgaatctctgattgatctgcaggaacttggaaaatatgaacagtacattaaatggccttggtacatttggcttggatttattgcaggattaattgcaattgtgatggtgacaattatgttatgttgtatgacatcatgttgttcttgtttaaaaggatgttgttcttgtggaagctgttgtaaatttgatgaagatgattctgaacctgtgttaaaaggagtgaaattgcattacaca

SEQ ID NO: 24 - RNA, 3819 nt, synthetic construct
  source 1..3819: mol_type = other RNA
atgttcgtgttcctggtgctgctgcctctggtgtccagccagtgtgtgaacctgaccaccagaacacagctgcctccagcctacaccaacagctttaccagaggcgtgtactaccccgacaaggtgttcagatccagcgtgctgcactctacccaggacctgttcctgcctttcttcagcaacgtgacctggttccacgccatccacgtgtccggcaccaatggcaccaagagattcgacaaccccgtgctgcccttcaacgacggggtgtactttgccagcaccgagaagtccaacatcatcagaggctggatcttcggcaccacactggacagcaagacccagagcctgctgatcgtgaacaacgccaccaacgtggtcatcaaagtgtgcgagttccagttctgcaacgaccccttcctgggcgtctactaccacaagaacaacaagagctggatggaaagcgagttccgggtgtacagcagcgccaacaactgcaccttcgagtacgtgtcccagcctttcctgatggacctggaaggcaagcagggcaacttcaagaacctgcgcgagttcgtgtttaagaacatcgacggctacttcaagatctacagcaagcacacccctatcaacctcgtgcgggatctgcctcagggcttctctgctctggaacccctggtggatctgcccatcggcatcaacatcacccggtttcagacactgctggccctgcacagaagctacctgacacctggcgatagcagcagcggatggacagctggtgccgccgcttactatgtgggctacctgcagcctagaaccttcctgctgaagtacaacgagaacggcaccatcaccgacgccgtggattgtgctctggatcctctgagcgagacaaagtgcaccctgaagtccttcaccgtggaaaagggcatctaccagaccagcaacttccgggtgcagcccaccgaatccatcgtgcggttccccaatatcaccaatctgtgccccttcggcgaggtgttcaatgccaccagattcgcctctgtgtacgcctggaaccggaagcggatcagcaattgcgtggccgactactccgtgctgtacaactccgccagcttcagcaccttcaagtgctacggcgtgtcccctaccaagctgaacgacctgtgcttcacaaacgtgtacgccgacagcttcgtgatccggggagatgaagtgcggcagattgcccctggacagacaggcaagatcgccgactacaactacaagctgcccgacgacttcaccggctgtgtgattgcctggaacagcaacaacctggactccaaagtcggcggcaactacaattacctgtaccggctgttccggaagtccaatctgaagcccttcgagcgggacatctccaccgagatctatcaggccggcagcaccccttgtaacggcgtggaaggcttcaactgctacttcccactgcagtcctacggctttcagcccacaaatggcgtgggctatcagccctacagagtggtggtgctgagcttcgaactgctgcatgcccctgccacagtgtgcggccctaagaaaagcaccaatctcgtgaagaacaaatgcgtgaacttcaacttcaacggcctgaccggcaccggcgtgctgacagagagcaacaagaagttcctgccattccagcagtttggccgggatatcgccgataccacagacgccgttagagatccccagacactggaaatcctggacatcaccccttgcagcttcggcggagtgtctgtgatcacccctggcaccaacaccagcaatcaggtggcagtgctgtaccaggacgtgaactgtaccgaagtgcccgtggccattcacgccgatcagctgacacctacatggcgggtgtactccaccggcagcaatgtgtttcagaccagagccggctgtctgatcggagccgagcacgtgaacaatagctacgagtgcgacatccccatcggcgctggaatctgcgccagctaccagacacagacaaacagccctcggagagccagaagcgtggccagccagagcatcattgcctacacaatgtctctgggcgccgagaacagcgtggcctactccaacaactctatcgctatccccaccaacttcaccatcagcgtgaccacagagatcctgcctgtgtccatgaccaagaccagcgtggactgcaccatgtacatctgcggcgattccaccgagtgctccaacctgctgctgcagtacggcagcttctgcacccagctgaatagagccctgacagggatcgccgtggaacaggacaagaacacccaagaggtgttcgcccaagtgaagcagatctacaagacccctcctatcaaggacttcggcggcttcaatttcagccagattctgcccgatcctagcaagcccagcaagcggagcttcatcgaggacctgctgttcaacaaagtgacactggccgacgccggcttcatcaagcagtatggcgattgtctgggcgacattgccgccagggatctgatttgcgcccagaagtttaacggactgacagtgctgcctcctctgctgaccgatgagatgatcgcccagtacacatctgccctgctggccggcacaatcacaagcggctggacatttggagcaggcgccgctctgcagatcccctttgctatgcagatggcctaccggttcaacggcatcggagtgacccagaatgtgctgtacgagaaccagaagctgatcgccaaccagttcaacagcgccatcggcaagatccaggacagcctgagcagcacagcaagcgccctgggaaagctgcaggacgtggtcaaccagaatgcccaggcactgaacaccctggtcaagcagctgtcctccaacttcggcgccatcagctctgtgctgaacgatatcctgagcagactggaccctcctgaggccgaggtgcagatcgacagactgatcacaggcagactgcagagcctccagacatacgtgacccagcagctgatcagagccgccgagattagagcctctgccaatctggccgccaccaagatgtctgagtgtgtgctgggccagagcaagagagtggacttttgcggcaagggctaccacctgatgagcttccctcagtctgcccctcacggcgtggtgtttctgcacgtgacatatgtgcccgctcaagagaagaatttcaccaccgctccagccatctgccacgacggcaaagcccactttcctagagaaggcgtgttcgtgtccaacggcacccattggttcgtgacacagcggaacttctacgagccccagatcatcaccaccgacaacaccttcgtgtctggcaactgcgacgtcgtgatcggcattgtgaacaataccgtgtacgaccctctgcagcccgagctggacagcttcaaagaggaactggacaagtactttaagaaccacacaagccccgacgtggacctgggcgatatcagcggaatcaatgccagcgtcgtgaacatccagaaagagatcgaccggctgaacgaggtggccaagaatctgaacgagagcctgatcgacctgcaagaactggggaagtacgagcagtacatcaagtggccctggtacatctggctgggctttatcgccggactgattgccatcgtgatggtcacaatcatgctgtgttgcatgaccagctgctgtagctgcctgaagggctgttgtagctgtggcagctgctgcaagttcgacgaggacgattctgagcccgtgctgaagggcgtgaaactgcactacaca

SEQ ID NO: 25 - protein, 41 aa, synthetic construct
GSGYIPEAPRDGQAYVRKDGEWVLLSTFLGRSLEVLFQGPG

SEQ ID NO: 26 - RNA, 123 nt, synthetic construct
  source 1..123: mol_type = other RNA
ggatctggttatattcctgaagctccaagagatgggcaagcttacgttcgtaaagatggcgaatgggtattactttctacctttttaggccggtccctggaggtgctgttccagggccccggc

SEQ ID NO: 27 - RNA, 47 nt, synthetic construct
  source 1..47: mol_type = other RNA
aactagtattcttctggtccccacagactcagagagaacccgccacc

SEQ ID NO: 28 - RNA, 4282 nt, synthetic construct
  source 1..4282: mol_type = other RNA
gggcgaactagtattcttctggtccccacagactcagagagaacccgccaccatgtttgtgtttcttgtgctgctgcctcttgtgtcttctcagtgtgtgaatttgacaacaagaacacagctgccaccagcttatacaaattcttttaccagaggagtgtattatcctgataaagtgtttagatcttctgtgctgcacagcacacaggacctgtttctgccattttttagcaatgtgacatggtttcatgcaattcatgtgtctggaacaaatggaacaaaaagatttgataatcctgtgctgccttttaatgatggagtgtattttgcttcaacagaaaagtcaaatattattagaggatggatttttggaacaacactggattctaaaacacagtctctgctgattgtgaataatgcaacaaatgtggtgattaaagtgtgtgaatttcagttttgtaatgatccttttctgggagtgtattatcacaaaaataataaatcttggatggaatctgaatttagagtgtattcctctgcaaataattgtacatttgaatatgtgtctcagccttttctgatggatctggaaggaaaacagggcaattttaaaaatctgagagaatttgtgtttaaaaatattgatggatattttaaaatttattctaaacacacaccaattaatttagtgagagatctgcctcagggattttctgctctggaacctctggtggatctgccaattggcattaatattacaagatttcagacactgctggctctgcacagatcttatctgacacctggagattcttcttctggatggacagccggagctgcagcttattatgtgggctatctgcagccaagaacatttctgctgaaatataatgaaaatggaacaattacagatgctgtggattgtgctctggatcctctgtctgaaacaaaatgtacattaaaatcttttacagtggaaaaaggcatttatcagacatctaattttagagtgcagccaacagaatctattgtgagatttccaaatattacaaatctgtgtccatttggagaagtgtttaatgcaacaagatttgcatctgtgtatgcatggaatagaaaaagaatttctaattgtgtggctgattattctgtgctgtataatagtgcttctttttccacatttaaatgttatggagtgtctccaacaaaattaaatgatttatgttttacaaatgtgtatgctgattcttttgtgatcagaggtgatgaagtgagacagattgcccccggacagacaggaaaaattgctgattacaattacaaactgcctgatgattttacaggatgtgtgattgcttggaattctaataatttagattctaaagtgggaggaaattacaattatctgtacagactgtttagaaaatcaaatctgaaaccttttgaaagagatatttcaacagaaatttatcaggctggatcaacaccttgtaatggagtggaaggatttaattgttattttccattacagagctatggatttcagccaaccaatggtgtgggatatcagccatatagagtggtggtgctgtcttttgaactgctgcatgcacctgcaacagtgtgtggacctaaaaaatctacaaatttagtgaaaaataaatgtgtgaattttaattttaatggattaacaggaacaggagtgctgacagaatctaataaaaaatttctgccttttcagcagtttggcagagatattgcagataccacagatgcagtgagagatcctcagacattagaaattctggatattacaccttgttcttttgggggtgtgtctgtgattacacctggaacaaatacatctaatcaggtggctgtgctgtatcaggatgtgaattgtacagaagtgccagtggcaattcatgcagatcagctgacaccaacatggagagtgtattctacaggatctaatgtgtttcagacaagagcaggatgtctgattggagcagaacatgtgaataattcttatgaatgtgatattccaattggagcaggcatttgtgcatcttatcagacacagacaaattccccaaggagagcaagatctgtggcatctcagtctattattgcatacaccatgtctctgggagcagaaaattctgtggcatattctaataattctattgctattccaacaaattttaccatttctgtgacaacagaaattttacctgtgtctatgacaaaaacatctgtggattgtaccatgtacatttgtggagattctacagaatgttctaatctgctgctgcagtatggatctttttgtacacagctgaatagagctttaacaggaattgctgtggaacaggataaaaatacacaggaagtgtttgctcaggtgaaacagatttacaaaacaccaccaattaaagattttggaggatttaattttagccagattctgcctgatccttctaaaccttctaaaagatcttttattgaagatctgctgtttaataaagtgacactggcagatgcaggatttattaaacagtatggagattgcctgggtgatattgctgcaagagatctgatttgtgctcagaaatttaatggactgacagtgctgcctcctctgctgacagatgaaatgattgctcagtacacatctgctttactggctggaacaattacaagcggatggacatttggagctggagctgctctgcagattccttttgcaatgcagatggcttacagatttaatggaattggagtgacacagaatgtgttatatgaaaatcagaaactgattgcaaatcagtttaattctgcaattggcaaaattcaggattctctgtcttctacagcttctgctctgggaaaactgcaggatgtggtgaatcagaatgcacaggcactgaatactctggtgaaacagctgtctagcaattttggggcaatttcttctgtgctgaatgatattctgtctagactggatcctcctgaagctgaagtgcagattgatagactgatcacaggaagactgcagtctctgcagacttatgtgacacagcagctgattagagctgctgaaattagagcttctgctaatctggctgctacaaaaatgtctgaatgtgtgctgggacagtcaaaaagagtggatttttgtggaaaaggatatcatctgatgtcttttccacagtctgctccacatggagtggtgtttttacatgtgacatatgtgccagcacaggaaaagaattttaccacagcaccagcaatttgtcatgatggaaaagcacattttccaagagaaggagtgtttgtgtctaatggaacacattggtttgtgacacagagaaatttttatgaacctcagattattacaacagataatacatttgtgtcaggaaattgtgatgtggtgattggaattgtgaataatacagtgtatgatccactgcagccagaactggattcttttaaagaagaactggataaatattttaaaaatcacacatctcctgatgtggatttaggagatatttctggaatcaatgcatctgtggtgaatattcagaaagaaattgatagactgaatgaagtggccaaaaatctgaatgaatctctgattgatctgcaggaacttggaaaatatgaacagtacattaaatggccttggtacatttggcttggatttattgcaggattaattgcaattgtgatggtgacaattatgttatgttgtatgacatcatgttgttcttgtttaaaaggatgttgttcttgtggaagctgttgtaaatttgatgaagatgattctgaacctgtgttaaaaggagtgaaattgcattacacatgatgactcgagctggtactgcatgcacgcaatgctagctgcccctttcccgtcctgggtaccccgagtctcccccgacctcgggtcccaggtatgctcccacctccacctgccccactcaccacctctgctagttccagacacctcccaagcacgcagcaatgcagctcaaaacgcttagcctagccacacccccacgggaaacagcagtgattaacctttagcaataaacgaaagtttaactaagctatactaaccccagggttggtcaatttcgtgccagccacaccctggagctagcaaaaaaaaaaaaaaaaaaaaaaaaaaaaaagcatatgactaaaaaaaaaaaaaaaaaaaaaaaaaaaaaaaaaaaaaaaaaaaaaaaaaaaaaaaaaaaaaaaaaaaaaa

SEQ ID NO: 29 - RNA, 4282 nt, synthetic construct
  source 1..4282: mol_type = other RNA
gggcgaactagtattcttctggtccccacagactcagagagaacccgccaccatgttcgtgttcctggtgctgctgcctctggtgtccagccagtgtgtgaacctgaccaccagaacacagctgcctccagcctacaccaacagctttaccagaggcgtgtactaccccgacaaggtgttcagatccagcgtgctgcactctacccaggacctgttcctgcctttcttcagcaacgtgacctggttccacgccatccacgtgtccggcaccaatggcaccaagagattcgacaaccccgtgctgcccttcaacgacggggtgtactttgccagcaccgagaagtccaacatcatcagaggctggatcttcggcaccacactggacagcaagacccagagcctgctgatcgtgaacaacgccaccaacgtggtcatcaaagtgtgcgagttccagttctgcaacgaccccttcctgggcgtctactaccacaagaacaacaagagctggatggaaagcgagttccgggtgtacagcagcgccaacaactgcaccttcgagtacgtgtcccagcctttcctgatggacctggaaggcaagcagggcaacttcaagaacctgcgcgagttcgtgtttaagaacatcgacggctacttcaagatctacagcaagcacacccctatcaacctcgtgcgggatctgcctcagggcttctctgctctggaacccctggtggatctgcccatcggcatcaacatcacccggtttcagacactgctggccctgcacagaagctacctgacacctggcgatagcagcagcggatggacagctggtgccgccgcttactatgtgggctacctgcagcctagaaccttcctgctgaagtacaacgagaacggcaccatcaccgacgccgtggattgtgctctggatcctctgagcgagacaaagtgcaccctgaagtccttcaccgtggaaaagggcatctaccagaccagcaacttccgggtgcagcccaccgaatccatcgtgcggttccccaatatcaccaatctgtgccccttcggcgaggtgttcaatgccaccagattcgcctctgtgtacgcctggaaccggaagcggatcagcaattgcgtggccgactactccgtgctgtacaactccgccagcttcagcaccttcaagtgctacggcgtgtcccctaccaagctgaacgacctgtgcttcacaaacgtgtacgccgacagcttcgtgatccggggagatgaagtgcggcagattgcccctggacagacaggcaagatcgccgactacaactacaagctgcccgacgacttcaccggctgtgtgattgcctggaacagcaacaacctggactccaaagtcggcggcaactacaattacctgtaccggctgttccggaagtccaatctgaagcccttcgagcgggacatctccaccgagatctatcaggccggcagcaccccttgtaacggcgtggaaggcttcaactgctacttcccactgcagtcctacggctttcagcccacaaatggcgtgggctatcagccctacagagtggtggtgctgagcttcgaactgctgcatgcccctgccacagtgtgcggccctaagaaaagcaccaatctcgtgaagaacaaatgcgtgaacttcaacttcaacggcctgaccggcaccggcgtgctgacagagagcaacaagaagttcctgccattccagcagtttggccgggatatcgccgataccacagacgccgttagagatccccagacactggaaatcctggacatcaccccttgcagcttcggcggagtgtctgtgatcacccctggcaccaacaccagcaatcaggtggcagtgctgtaccaggacgtgaactgtaccgaagtgcccgtggccattcacgccgatcagctgacacctacatggcgggtgtactccaccggcagcaatgtgtttcagaccagagccggctgtctgatcggagccgagcacgtgaacaatagctacgagtgcgacatccccatcggcgctggaatctgcgccagctaccagacacagacaaacagccctcggagagccagaagcgtggccagccagagcatcattgcctacacaatgtctctgggcgccgagaacagcgtggcctactccaacaactctatcgctatccccaccaacttcaccatcagcgtgaccacagagatcctgcctgtgtccatgaccaagaccagcgtggactgcaccatgtacatctgcggcgattccaccgagtgctccaacctgctgctgcagtacggcagcttctgcacccagctgaatagagccctgacagggatcgccgtggaacaggacaagaacacccaagaggtgttcgcccaagtgaagcagatctacaagacccctcctatcaaggacttcggcggcttcaatttcagccagattctgcccgatcctagcaagcccagcaagcggagcttcatcgaggacctgctgttcaacaaagtgacactggccgacgccggcttcatcaagcagtatggcgattgtctgggcgacattgccgccagggatctgatttgcgcccagaagtttaacggactgacagtgctgcctcctctgctgaccgatgagatgatcgcccagtacacatctgccctgctggccggcacaatcacaagcggctggacatttggagcaggcgccgctctgcagatcccctttgctatgcagatggcctaccggttcaacggcatcggagtgacccagaatgtgctgtacgagaaccagaagctgatcgccaaccagttcaacagcgccatcggcaagatccaggacagcctgagcagcacagcaagcgccctgggaaagctgcaggacgtggtcaaccagaatgcccaggcactgaacaccctggtcaagcagctgtcctccaacttcggcgccatcagctctgtgctgaacgatatcctgagcagactggaccctcctgaggccgaggtgcagatcgacagactgatcacaggcagactgcagagcctccagacatacgtgacccagcagctgatcagagccgccgagattagagcctctgccaatctggccgccaccaagatgtctgagtgtgtgctgggccagagcaagagagtggacttttgcggcaagggctaccacctgatgagcttccctcagtctgcccctcacggcgtggtgtttctgcacgtgacatatgtgcccgctcaagagaagaatttcaccaccgctccagccatctgccacgacggcaaagcccactttcctagagaaggcgtgttcgtgtccaacggcacccattggttcgtgacacagcggaacttctacgagccccagatcatcaccaccgacaacaccttcgtgtctggcaactgcgacgtcgtgatcggcattgtgaacaataccgtgtacgaccctctgcagcccgagctggacagcttcaaagaggaactggacaagtactttaagaaccacacaagccccgacgtggacctgggcgatatcagcggaatcaatgccagcgtcgtgaacatccagaaagagatcgaccggctgaacgaggtggccaagaatctgaacgagagcctgatcgacctgcaagaactggggaagtacgagcagtacatcaagtggccctggtacatctggctgggctttatcgccggactgattgccatcgtgatggtcacaatcatgctgtgttgcatgaccagctgctgtagctgcctgaagggctgttgtagctgtggcagctgctgcaagttcgacgaggacgattctgagcccgtgctgaagggcgtgaaactgcactacacatgatgactcgagctggtactgcatgcacgcaatgctagctgcccctttcccgtcctgggtaccccgagtctcccccgacctcgggtcccaggtatgctcccacctccacctgccccactcaccacctctgctagttccagacacctcccaagcacgcagcaatgcagctcaaaacgcttagcctagccacacccccacgggaaacagcagtgattaacctttagcaataaacgaaagtttaactaagctatactaaccccagggttggtcaatttcgtgccagccacaccctggagctagcaaaaaaaaaaaaaaaaaaaaaaaaaaaaaagcatatgactaaaaaaaaaaaaaaaaaaaaaaaaaaaaaaaaaaaaaaaaaaaaaaaaaaaaaaaaaaaaaaaaaaaaaa

SEQ ID NO: 30 - RNA, 1261 nt, synthetic construct
  source 1..1261: mol_type = other RNA
gggcgaactagtattcttctggtccccacagactcagagagaacccgccaccatgtttgtgtttcttgtgctgctgcctcttgtgtcttctcagtgtgtggtgagatttccaaatattacaaatctgtgtccatttggagaagtgtttaatgcaacaagatttgcatctgtgtatgcatggaatagaaaaagaatttctaattgtgtggctgattattctgtgctgtataatagtgcttctttttccacatttaaatgttatggagtgtctccaacaaaattaaatgatttatgttttacaaatgtgtatgctgattcttttgtgatcagaggtgatgaagtgagacagattgcccccggacagacaggaaaaattgctgattacaattacaaactgcctgatgattttacaggatgtgtgattgcttggaattctaataatttagattctaaagtgggaggaaattacaattatctgtacagactgtttagaaaatcaaatctgaaaccttttgaaagagatatttcaacagaaatttatcaggctggatcaacaccttgtaatggagtggaaggatttaattgttattttccattacagagctatggatttcagccaaccaatggtgtgggatatcagccatatagagtggtggtgctgtcttttgaactgctgcatgcacctgcaacagtgtgtggacctaaaggctcccccggctccggctccggatctggttatattcctgaagctccaagagatgggcaagcttacgttcgtaaagatggcgaatgggtattactttctacctttttaggccggtccctggaggtgctgttccagggccccggctgatgactcgagctggtactgcatgcacgcaatgctagctgcccctttcccgtcctgggtaccccgagtctcccccgacctcgggtcccaggtatgctcccacctccacctgccccactcaccacctctgctagttccagacacctcccaagcacgcagcaatgcagctcaaaacgcttagcctagccacacccccacgggaaacagcagtgattaacctttagcaataaacgaaagtttaactaagctatactaaccccagggttggtcaatttcgtgccagccacaccctggagctagcaaaaaaaaaaaaaaaaaaaaaaaaaaaaaagcatatgactaaaaaaaaaaaaaaaaaaaaaaaaaaaaaaaaaaaaaaaaaaaaaaaaaaaaaaaaaaaaaaaaaaaaaa

SEQ ID NO: 31 - RNA, 4283 nt, synthetic construct
  source 1..4283: mol_type = other RNA
agaataaactagtattcttctggtccccacagactcagagagaacccgccaccatgtttgtgtttcttgtgctgctgcctcttgtgtcttctcagtgtgtgaatttgacaacaagaacacagctgccaccagcttatacaaattcttttaccagaggagtgtattatcctgataaagtgtttagatcttctgtgctgcacagcacacaggacctgtttctgccattttttagcaatgtgacatggtttcatgcaattcatgtgtctggaacaaatggaacaaaaagatttgataatcctgtgctgccttttaatgatggagtgtattttgcttcaacagaaaagtcaaatattattagaggatggatttttggaacaacactggattctaaaacacagtctctgctgattgtgaataatgcaacaaatgtggtgattaaagtgtgtgaatttcagttttgtaatgatccttttctgggagtgtattatcacaaaaataataaatcttggatggaatctgaatttagagtgtattcctctgcaaataattgtacatttgaatatgtgtctcagccttttctgatggatctggaaggaaaacagggcaattttaaaaatctgagagaatttgtgtttaaaaatattgatggatattttaaaatttattctaaacacacaccaattaatttagtgagagatctgcctcagggattttctgctctggaacctctggtggatctgccaattggcattaatattacaagatttcagacactgctggctctgcacagatcttatctgacacctggagattcttcttctggatggacagccggagctgcagcttattatgtgggctatctgcagccaagaacatttctgctgaaatataatgaaaatggaacaattacagatgctgtggattgtgctctggatcctctgtctgaaacaaaatgtacattaaaatcttttacagtggaaaaaggcatttatcagacatctaattttagagtgcagccaacagaatctattgtgagatttccaaatattacaaatctgtgtccatttggagaagtgtttaatgcaacaagatttgcatctgtgtatgcatggaatagaaaaagaatttctaattgtgtggctgattattctgtgctgtataatagtgcttctttttccacatttaaatgttatggagtgtctccaacaaaattaaatgatttatgttttacaaatgtgtatgctgattcttttgtgatcagaggtgatgaagtgagacagattgcccccggacagacaggaaaaattgctgattacaattacaaactgcctgatgattttacaggatgtgtgattgcttggaattctaataatttagattctaaagtgggaggaaattacaattatctgtacagactgtttagaaaatcaaatctgaaaccttttgaaagagatatttcaacagaaatttatcaggctggatcaacaccttgtaatggagtggaaggatttaattgttattttccattacagagctatggatttcagccaaccaatggtgtgggatatcagccatatagagtggtggtgctgtcttttgaactgctgcatgcacctgcaacagtgtgtggacctaaaaaatctacaaatttagtgaaaaataaatgtgtgaattttaattttaatggattaacaggaacaggagtgctgacagaatctaataaaaaatttctgccttttcagcagtttggcagagatattgcagataccacagatgcagtgagagatcctcagacattagaaattctggatattacaccttgttcttttgggggtgtgtctgtgattacacctggaacaaatacatctaatcaggtggctgtgctgtatcaggatgtgaattgtacagaagtgccagtggcaattcatgcagatcagctgacaccaacatggagagtgtattctacaggatctaatgtgtttcagacaagagcaggatgtctgattggagcagaacatgtgaataattcttatgaatgtgatattccaattggagcaggcatttgtgcatcttatcagacacagacaaattccccaaggagagcaagatctgtggcatctcagtctattattgcatacaccatgtctctgggagcagaaaattctgtggcatattctaataattctattgctattccaacaaattttaccatttctgtgacaacagaaattttacctgtgtctatgacaaaaacatctgtggattgtaccatgtacatttgtggagattctacagaatgttctaatctgctgctgcagtatggatctttttgtacacagctgaatagagctttaacaggaattgctgtggaacaggataaaaatacacaggaagtgtttgctcaggtgaaacagatttacaaaacaccaccaattaaagattttggaggatttaattttagccagattctgcctgatccttctaaaccttctaaaagatcttttattgaagatctgctgtttaataaagtgacactggcagatgcaggatttattaaacagtatggagattgcctgggtgatattgctgcaagagatctgatttgtgctcagaaatttaatggactgacagtgctgcctcctctgctgacagatgaaatgattgctcagtacacatctgctttactggctggaacaattacaagcggatggacatttggagctggagctgctctgcagattccttttgcaatgcagatggcttacagatttaatggaattggagtgacacagaatgtgttatatgaaaatcagaaactgattgcaaatcagtttaattctgcaattggcaaaattcaggattctctgtcttctacagcttctgctctgggaaaactgcaggatgtggtgaatcagaatgcacaggcactgaatactctggtgaaacagctgtctagcaattttggggcaatttcttctgtgctgaatgatattctgtctagactggatcctcctgaagctgaagtgcagattgatagactgatcacaggaagactgcagtctctgcagacttatgtgacacagcagctgattagagctgctgaaattagagcttctgctaatctggctgctacaaaaatgtctgaatgtgtgctgggacagtcaaaaagagtggatttttgtggaaaaggatatcatctgatgtcttttccacagtctgctccacatggagtggtgtttttacatgtgacatatgtgccagcacaggaaaagaattttaccacagcaccagcaatttgtcatgatggaaaagcacattttccaagagaaggagtgtttgtgtctaatggaacacattggtttgtgacacagagaaatttttatgaacctcagattattacaacagataatacatttgtgtcaggaaattgtgatgtggtgattggaattgtgaataatacagtgtatgatccactgcagccagaactggattcttttaaagaagaactggataaatattttaaaaatcacacatctcctgatgtggatttaggagatatttctggaatcaatgcatctgtggtgaatattcagaaagaaattgatagactgaatgaagtggccaaaaatctgaatgaatctctgattgatctgcaggaacttggaaaatatgaacagtacattaaatggccttggtacatttggcttggatttattgcaggattaattgcaattgtgatggtgacaattatgttatgttgtatgacatcatgttgttcttgtttaaaaggatgttgttcttgtggaagctgttgtaaatttgatgaagatgattctgaacctgtgttaaaaggagtgaaattgcattacacatgatgactcgagctggtactgcatgcacgcaatgctagctgcccctttcccgtcctgggtaccccgagtctcccccgacctcgggtcccaggtatgctcccacctccacctgccccactcaccacctctgctagttccagacacctcccaagcacgcagcaatgcagctcaaaacgcttagcctagccacacccccacgggaaacagcagtgattaacctttagcaataaacgaaagtttaactaagctatactaaccccagggttggtcaatttcgtgccagccacaccctggagctagcaaaaaaaaaaaaaaaaaaaaaaaaaaaaaagcatatgactaaaaaaaaaaaaaaaaaaaaaaaaaaaaaaaaaaaaaaaaaaaaaaaaaaaaaaaaaaaaaaaaaaaaaa

SEQ ID NO: 32 - RNA, 1262 nt, synthetic construct
  source 1..1262: mol_type = other RNA
agaataaactagtattcttctggtccccacagactcagagagaacccgccaccatgtttgtgtttcttgtgctgctgcctcttgtgtcttctcagtgtgtggtgagatttccaaatattacaaatctgtgtccatttggagaagtgtttaatgcaacaagatttgcatctgtgtatgcatggaatagaaaaagaatttctaattgtgtggctgattattctgtgctgtataatagtgcttctttttccacatttaaatgttatggagtgtctccaacaaaattaaatgatttatgttttacaaatgtgtatgctgattcttttgtgatcagaggtgatgaagtgagacagattgcccccggacagacaggaaaaattgctgattacaattacaaactgcctgatgattttacaggatgtgtgattgcttggaattctaataatttagattctaaagtgggaggaaattacaattatctgtacagactgtttagaaaatcaaatctgaaaccttttgaaagagatatttcaacagaaatttatcaggctggatcaacaccttgtaatggagtggaaggatttaattgttattttccattacagagctatggatttcagccaaccaatggtgtgggatatcagccatatagagtggtggtgctgtcttttgaactgctgcatgcacctgcaacagtgtgtggacctaaaggctcccccggctccggctccggatctggttatattcctgaagctccaagagatgggcaagcttacgttcgtaaagatggcgaatgggtattactttctacctttttaggccggtccctggaggtgctgttccagggccccggctgatgactcgagctggtactgcatgcacgcaatgctagctgcccctttcccgtcctgggtaccccgagtctcccccgacctcgggtcccaggtatgctcccacctccacctgccccactcaccacctctgctagttccagacacctcccaagcacgcagcaatgcagctcaaaacgcttagcctagccacacccccacgggaaacagcagtgattaacctttagcaataaacgaaagtttaactaagctatactaaccccagggttggtcaatttcgtgccagccacaccctggagctagcaaaaaaaaaaaaaaaaaaaaaaaaaaaaaagcatatgactaaaaaaaaaaaaaaaaaaaaaaaaaaaaaaaaaaaaaaaaaaaaaaaaaaaaaaaaaaaaaaaaaaaaaa

SEQ ID NO: 33 - RNA, 11917 nt, synthetic construct
  source 1..11917: mol_type = other RNA
gatgggcggcgcatgagagaagcccagaccaattacctacccaaaatggagaaagttcacgttgacatcgaggaagacagcccattcctcagagctttgcagcggagcttcccgcagtttgaggtagaagccaagcaggtcactgataatgaccatgctaatgccagagcgttttcgcatctggcttcaaaactgatcgaaacggaggtggacccatccgacacgatccttgacattggaagtgcgcccgcccgcagaatgtattctaagcacaagtatcattgtatctgtccgatgagatgtgcggaagatccggacagattgtataagtatgcaactaagctgaagaaaaactgtaaggaaataactgataaggaattggacaagaaaatgaaggagctcgccgccgtcatgagcgaccctgacctggaaactgagactatgtgcctccacgacgacgagtcgtgtcgctacgaagggcaagtcgctgtttaccaggatgtatacgcggttgacggaccgacaagtctctatcaccaagccaataagggagttagagtcgcctactggataggctttgacaccaccccttttatgtttaagaacttggctggagcatatccatcatactctaccaactgggccgacgaaaccgtgttaacggctcgtaacataggcctatgcagctctgacgttatggagcggtcacgtagagggatgtccattcttagaaagaagtatttgaaaccatccaacaatgttctattctctgttggctcgaccatctaccacgaaaagagggacttactgaggagctggcacctgccgtctgtatttcacttacgtggcaagcaaaattacacatgtcggtgtgagactatagttagttgcgacgggtacgtcgttaaaagaatagctatcagtccaggcctgtatgggaagccttcaggctatgctgctacgatgcaccgcgagggattcttgtgctgcaaagtgacagacacattgaacggggagagggtctcttttcccgtgtgcacgtatgtgccagctacattgtgtgaccaaatgactggcatactggcaacagatgtcagtgcggacgacgcgcaaaaactgctggttgggctcaaccagcgtatagtcgtcaacggtcgcacccagagaaacaccaataccatgaaaaattaccttttgcccgtagtggcccaggcatttgctaggtgggcaaaggaatataaggaagatcaagaagatgaaaggccactaggactacgagatagacagttagtcatggggtgttgttgggcttttagaaggcacaagataacatctatttataagcgcccggatacccaaaccatcatcaaagtgaacagcgatttccactcattcgtgctgcccaggataggcagtaacacattggagatcgggctgagaacaagaatcaggaaaatgttagaggagcacaaggagccgtcacctctcattaccgccgaggacgtacaagaagctaagtgcgcagccgatgaggctaaggaggtgcgtgaagccgaggagttgcgcgcagctctaccacctttggcagctgatgttgaggagcccactctggaagccgatgtcgacttgatgttacaagaggctggggccggctcagtggagacacctcgtggcttgataaaggttaccagctacgctggcgaggacaagatcggctcttacgctgtgctttctccgcaggctgtactcaagagtgaaaaattatcttgcatccaccctctcgctgaacaagtcatagtgataacacactctggccgaaaagggcgttatgccgtggaaccataccatggtaaagtagtggtgccagagggacatgcaatacccgtccaggactttcaagctctgagtgaaagtgccaccattgtgtacaacgaacgtgagttcgtaaacaggtacctgcaccatattgccacacatggaggagcgctgaacactgatgaagaatattacaaaactgtcaagcccagcgagcacgacggcgaatacctgtacgacatcgacaggaaacagtgcgtcaagaaagagctagtcactgggctagggctcacaggcgagctggtcgatcctcccttccatgaattcgcctacgagagtctgagaacacgaccagccgctccttaccaagtaccaaccataggggtgtatggcgtgccaggatcaggcaagtctggcatcattaaaagcgcagtcaccaaaaaagatctagtggtgagcgccaagaaagaaaactgtgcagaaattataagggacgtcaagaaaatgaaagggctggacgtcaatgccagaactgtggactcagtgctcttgaatggatgcaaacaccccgtagagaccctgtatattgacgaggcttttgcttgtcatgcaggtactctcagagcgctcatagccattataagacctaaaaaggcagtgctctgcggagatcccaaacagtgcggtttttttaacatgatgtgcctgaaagtgcattttaaccacgagatttgcacacaagtcttccacaaaagcatctctcgccgttgcactaaatctgtgacttcggtcgtctcaaccttgttttacgacaaaaaaatgagaacgacgaatccgaaagagactaagattgtgattgacactaccggcagtaccaaacctaagcaggacgatctcattctcacttgtttcagagggtgggtgaagcagttgcaaatagattacaaaggcaacgaaataatgacggcagctgcctctcaagggctgacccgtaaaggtgtgtatgccgttcggtacaaggtgaatgaaaatcctctgtacgcacccacctcagaacatgtgaacgtcctactgacccgcacggaggaccgcatcgtgtggaaaacactagccggcgacccatggataaaaacactgactgccaagtaccctgggaatttcactgccacgatagaggagtggcaagcagagcatgatgccatcatgaggcacatcttggagagaccggaccctaccgacgtcttccagaataaggcaaacgtgtgttgggccaaggctttagtgccggtgctgaagaccgctggcatagacatgaccactgaacaatggaacactgtggattattttgaaacggacaaagctcactcagcagagatagtattgaaccaactatgcgtgaggttctttggactcgatctggactccggtctattttctgcacccactgttccgttatccattaggaataatcactgggataactccccgtcgcctaacatgtacgggctgaataaagaagtggtccgtcagctctctcgcaggtacccacaactgcctcgggcagttgccactggtagagtctatgacatgaacactggtacactgcgcaattatgatccgcgcataaacctagtacctgtaaacagaagactgcctcatgctttagtcctccaccataatgaacacccacagagtgacttttcttcattcgtcagcaaattgaagggcagaactgtcctggtggtcggggaaaagttgtccgtcccaggcaaaatggttgactggttgtcagaccggcctgaggctaccttcagagctcggctggatttaggcatcccaggtgatgtgcccaaatatgacataatatttgttaatgtgaggaccccatataaataccatcactatcagcagtgtgaagaccatgccattaagctaagcatgttgaccaagaaagcatgtctgcatctgaatcccggcggaacctgtgtcagcataggttatggttacgctgacagggccagcgaaagcatcattggtgctatagcgcggcagttcaagttttcccgagtatgcaaaccgaaatcctcacttgaggagacggaagttctgtttgtattcattgggtacgatcgcaaggcccgtacgcacaatccttacaagctatcatcaaccttgaccaacatttatacaggttccagactccacgaagccggatgtgcaccctcatatcatgtggtgcgaggggatattgccacggccaccgaaggagtgattataaatgctgctaacagcaaaggacaacctggcggaggggtgtgcggagcgctgtataagaaattcccggaaagtttcgatttacagccgatcgaagtaggaaaagcgcgactggtcaaaggtgcagctaaacatatcattcatgccgtaggaccaaacttcaacaaagtttcggaggttgaaggtgacaaacagttggcagaggcttatgagtccatcgctaagattgtcaacgataacaattacaagtcagtagcgattccactgttgtccaccggcatcttttccgggaacaaagatcgactaacccaatcattgaaccatttgctgacagctttagacaccactgatgcagatgtagccatatactgcagggacaagaaatgggaaatgactctcaaggaagcagtggctaggagagaagcagtggaggagatatgcatatccgacgattcttcagtgacagaacctgatgcagagctggtgagggtgcatcccaagagttctttggctggaaggaagggctacagcacaagcgatggcaaaactttctcatatttggaagggaccaagtttcaccaggcggccaaggatatagcagaaattaatgccatgtggcccgttgcaacggaggccaatgagcaggtatgcatgtatatcctcggagaaagcatgagcagtattaggtcgaaatgccccgtcgaggagtcggaagcctccacaccacctagcacgctgccttgcttgtgcatccatgccatgactccagaaagagtacagcgcctaaaagcctcacgtccagaacaaattactgtgtgctcatcctttccattgccgaagtatagaatcactggtgtgcagaagatccaatgctcccagcctatattgttctcaccgaaagtgcctgcgtatattcatccaaggaagtatctcgtggaaacaccaccggtagacgagactccggagccatcggcagagaaccaatccacagaggggacacctgaacaaccaccacttataaccgaggatgagaccaggactagaacgcctgagccgatcatcatcgaagaagaagaagaagatagcataagtttgctgtcagatggcccgacccaccaggtgctgcaagtcgaggcagacattcacgggccgccctctgtatctagctcatcctggtccattcctcatgcatccgactttgatgtggacagtttatccatacttgacaccctggagggagctagcgtgaccagcggggcaacgtcagccgagactaactcttacttcgcaaagagtatggagtttctggcgcgaccggtgcctgcgcctcgaacagtattcaggaaccctccacatcccgctccgcgcacaagaacaccgtcacttgcacccagcagggcctgctccagaaccagcctagtttccaccccgccaggcgtgaatagggtgatcactagagaggagctcgaagcgcttaccccgtcacgcactcctagcaggtcggtctccagaaccagcctggtctccaacccgccaggcgtaaatagggtgattacaagagaggagtttgaggcgttcgtagcacaacaacaatgacggtttgatgcgggtgcatacatcttttcctccgacaccggtcaagggcatttacaacaaaaatcagtaaggcaaacggtgctatccgaagtggtgttggagaggaccgaattggagatttcgtatgccccgcgcctcgaccaagaaaaagaagaattactacgcaagaaattacagttaaatcccacacctgctaacagaagcagataccagtccaggaaggtggagaacatgaaagccataacagctagacgtattctgcaaggcctagggcattatttgaaggcagaaggaaaagtggagtgctaccgaaccctgcatcctgttcctttgtattcatctagtgtgaaccgtgccttttcaagccccaaggtcgcagtggaagcctgtaacgccatgttgaaagagaactttccgactgtggcttcttactgtattattccagagtacgatgcctatttggacatggttgacggagcttcatgctgcttagacactgccagtttttgccctgcaaagctgcgcagctttccaaagaaacactcctatttggaacccacaatacgatcggcagtgccttcagcgatccagaacacgctccagaacgtcctggcagctgccacaaaaagaaattgcaatgtcacgcaaatgagagaattgcccgtattggattcggcggcctttaatgtggaatgcttcaagaaatatgcgtgtaataatgaatattgggaaacgtttaaagaaaaccccatcaggcttactgaagaaaacgtggtaaattacattaccaaattaaaaggaccaaaagctgctgctctttttgcgaagacacataatttgaatatgttgcaggacataccaatggacaggtttgtaatggacttaaagagagacgtgaaagtgactccaggaacaaaacatactgaagaacggcccaaggtacaggtgatccaggctgccgatccgctagcaacagcgtatctgtgcggaatccaccgagagctggttaggagattaaatgcggtcctgcttccgaacattcatacactgtttgatatgtcggctgaagactttgacgctattatagccgagcacttccagcctggggattgtgttctggaaactgacatcgcgtcgtttgataaaagtgaggacgacgccatggctctgaccgcgttaatgattctggaagacttaggtgtggacgcagagctgttgacgctgattgaggcggctttcggcgaaatttcatcaatacatttgcccactaaaactaaatttaaattcggagccatgatgaaatctggaatgttcctcacactgtttgtgaacacagtcattaacattgtaatcgcaagcagagtgttgagagaacggctaaccggatcaccatgtgcagcattcattggagatgacaatatcgtgaaaggagtcaaatcggacaaattaatggcagacaggtgcgccacctggttgaatatggaagtcaagattatagatgctgtggtgggcgagaaagcgccttatttctgtggagggtttattttgtgtgactccgtgaccggcacagcgtgccgtgtggcagaccccctaaaaaggctgtttaagctaggcaaacctctggcagcagacgatgaacatgatgatgacaggagaagggcattgcatgaggagtcaacacgctggaaccgagtgggtattctttcagagctgtgcaaggcagtagaatcaaggtatgaaaccgtaggaacttccatcatagttatggccatgactactctagctagcagtgttaaatcattcagctacctgagaggggcccctataactctctacggctaacctgaatggactacgacatagtctagtccgccaagactagtatgtttgtgtttcttgtgctgctgcctcttgtgtcttctcagtgtgtgaatttgacaacaagaacacagctgccaccagcttatacaaattcttttaccagaggagtgtattatcctgataaagtgtttagatcttctgtgctgcacagcacacaggacctgtttctgccattttttagcaatgtgacatggtttcatgcaattcatgtgtctggaacaaatggaacaaaaagatttgataatcctgtgctgccttttaatgatggagtgtattttgcttcaacagaaaagtcaaatattattagaggatggatttttggaacaacactggattctaaaacacagtctctgctgattgtgaataatgcaacaaatgtggtgattaaagtgtgtgaatttcagttttgtaatgatccttttctgggagtgtattatcacaaaaataataaatcttggatggaatctgaatttagagtgtattcctctgcaaataattgtacatttgaatatgtgtctcagccttttctgatggatctggaaggaaaacagggcaattttaaaaatctgagagaatttgtgtttaaaaatattgatggatattttaaaatttattctaaacacacaccaattaatttagtgagagatctgcctcagggattttctgctctggaacctctggtggatctgccaattggcattaatattacaagatttcagacactgctggctctgcacagatcttatctgacacctggagattcttcttctggatggacagccggagctgcagcttattatgtgggctatctgcagccaagaacatttctgctgaaatataatgaaaatggaacaattacagatgctgtggattgtgctctggatcctctgtctgaaacaaaatgtacattaaaatcttttacagtggaaaaaggcatttatcagacatctaattttagagtgcagccaacagaatctattgtgagatttccaaatattacaaatctgtgtccatttggagaagtgtttaatgcaacaagatttgcatctgtgtatgcatggaatagaaaaagaatttctaattgtgtggctgattattctgtgctgtataatagtgcttctttttccacatttaaatgttatggagtgtctccaacaaaattaaatgatttatgttttacaaatgtgtatgctgattcttttgtgatcagaggtgatgaagtgagacagattgcccccggacagacaggaaaaattgctgattacaattacaaactgcctgatgattttacaggatgtgtgattgcttggaattctaataatttagattctaaagtgggaggaaattacaattatctgtacagactgtttagaaaatcaaatctgaaaccttttgaaagagatatttcaacagaaatttatcaggctggatcaacaccttgtaatggagtggaaggatttaattgttattttccattacagagctatggatttcagccaaccaatggtgtgggatatcagccatatagagtggtggtgctgtcttttgaactgctgcatgcacctgcaacagtgtgtggacctaaaaaatctacaaatttagtgaaaaataaatgtgtgaattttaattttaatggattaacaggaacaggagtgctgacagaatctaataaaaaatttctgccttttcagcagtttggcagagatattgcagataccacagatgcagtgagagatcctcagacattagaaattctggatattacaccttgttcttttgggggtgtgtctgtgattacacctggaacaaatacatctaatcaggtggctgtgctgtatcaggatgtgaattgtacagaagtgccagtggcaattcatgcagatcagctgacaccaacatggagagtgtattctacaggatctaatgtgtttcagacaagagcaggatgtctgattggagcagaacatgtgaataattcttatgaatgtgatattccaattggagcaggcatttgtgcatcttatcagacacagacaaattccccaaggagagcaagatctgtggcatctcagtctattattgcatacaccatgtctctgggagcagaaaattctgtggcatattctaataattctattgctattccaacaaattttaccatttctgtgacaacagaaattttacctgtgtctatgacaaaaacatctgtggattgtaccatgtacatttgtggagattctacagaatgttctaatctgctgctgcagtatggatctttttgtacacagctgaatagagctttaacaggaattgctgtggaacaggataaaaatacacaggaagtgtttgctcaggtgaaacagatttacaaaacaccaccaattaaagattttggaggatttaattttagccagattctgcctgatccttctaaaccttctaaaagatcttttattgaagatctgctgtttaataaagtgacactggcagatgcaggatttattaaacagtatggagattgcctgggtgatattgctgcaagagatctgatttgtgctcagaaatttaatggactgacagtgctgcctcctctgctgacagatgaaatgattgctcagtacacatctgctttactggctggaacaattacaagcggatggacatttggagctggagctgctctgcagattccttttgcaatgcagatggcttacagatttaatggaattggagtgacacagaatgtgttatatgaaaatcagaaactgattgcaaatcagtttaattctgcaattggcaaaattcaggattctctgtcttctacagcttctgctctgggaaaactgcaggatgtggtgaatcagaatgcacaggcactgaatactctggtgaaacagctgtctagcaattttggggcaatttcttctgtgctgaatgatattctgtctagactggatcctcctgaagctgaagtgcagattgatagactgatcacaggaagactgcagtctctgcagacttatgtgacacagcagctgattagagctgctgaaattagagcttctgctaatctggctgctacaaaaatgtctgaatgtgtgctgggacagtcaaaaagagtggatttttgtggaaaaggatatcatctgatgtcttttccacagtctgctccacatggagtggtgtttttacatgtgacatatgtgccagcacaggaaaagaattttaccacagcaccagcaatttgtcatgatggaaaagcacattttccaagagaaggagtgtttgtgtctaatggaacacattggtttgtgacacagagaaatttttatgaacctcagattattacaacagataatacatttgtgtcaggaaattgtgatgtggtgattggaattgtgaataatacagtgtatgatccactgcagccagaactggattcttttaaagaagaactggataaatattttaaaaatcacacatctcctgatgtggatttaggagatatttctggaatcaatgcatctgtggtgaatattcagaaagaaattgatagactgaatgaagtggccaaaaatctgaatgaatctctgattgatctgcaggaacttggaaaatatgaacagtacattaaatggccttggtacatttggcttggatttattgcaggattaattgcaattgtgatggtgacaattatgttatgttgtatgacatcatgttgttcttgtttaaaaggatgttgttcttgtggaagctgttgtaaatttgatgaagatgattctgaacctgtgttaaaaggagtgaaattgcattacacatgatgactcgagctggtactgcatgcacgcaatgctagctgcccctttcccgtcctgggtaccccgagtctcccccgacctcgggtcccaggtatgctcccacctccacctgccccactcaccacctctgctagttccagacacctcccaagcacgcagcaatgcagctcaaaacgcttagcctagccacacccccacgggaaacagcagtgattaacctttagcaataaacgaaagtttaactaagctatactaaccccagggttggtcaatttcgtgccagccacaccgcggccgcatgaatacagcagcaattggcaagctgcttacatagaactcgcggcgattggcatgccgccttaaaatttttattttattttttcttttcttttccgaatcggattttgtttttaatatttcaaaaaaaaaaaaaaaaaaaaaaaaaaaaaagcatatgactaaaaaaaaaaaaaaaaaaaaaaaaaaaaaaaaaaaaaaaaaaaaaaaaaaaaaaaaaaaaaaaaaaaaaa

SEQ ID NO: 34 - RNA, 11917 nt, synthetic construct
  source 1..11917: mol_type = other RNA
gatgggcggcgcatgagagaagcccagaccaattacctacccaaaatggagaaagttcacgttgacatcgaggaagacagcccattcctcagagctttgcagcggagcttcccgcagtttgaggtagaagccaagcaggtcactgataatgaccatgctaatgccagagcgttttcgcatctggcttcaaaactgatcgaaacggaggtggacccatccgacacgatccttgacattggaagtgcgcccgcccgcagaatgtattctaagcacaagtatcattgtatctgtccgatgagatgtgcggaagatccggacagattgtataagtatgcaactaagctgaagaaaaactgtaaggaaataactgataaggaattggacaagaaaatgaaggagctcgccgccgtcatgagcgaccctgacctggaaactgagactatgtgcctccacgacgacgagtcgtgtcgctacgaagggcaagtcgctgtttaccaggatgtatacgcggttgacggaccgacaagtctctatcaccaagccaataagggagttagagtcgcctactggataggctttgacaccaccccttttatgtttaagaacttggctggagcatatccatcatactctaccaactgggccgacgaaaccgtgttaacggctcgtaacataggcctatgcagctctgacgttatggagcggtcacgtagagggatgtccattcttagaaagaagtatttgaaaccatccaacaatgttctattctctgttggctcgaccatctaccacgaaaagagggacttactgaggagctggcacctgccgtctgtatttcacttacgtggcaagcaaaattacacatgtcggtgtgagactatagttagttgcgacgggtacgtcgttaaaagaatagctatcagtccaggcctgtatgggaagccttcaggctatgctgctacgatgcaccgcgagggattcttgtgctgcaaagtgacagacacattgaacggggagagggtctcttttcccgtgtgcacgtatgtgccagctacattgtgtgaccaaatgactggcatactggcaacagatgtcagtgcggacgacgcgcaaaaactgctggttgggctcaaccagcgtatagtcgtcaacggtcgcacccagagaaacaccaataccatgaaaaattaccttttgcccgtagtggcccaggcatttgctaggtgggcaaaggaatataaggaagatcaagaagatgaaaggccactaggactacgagatagacagttagtcatggggtgttgttgggcttttagaaggcacaagataacatctatttataagcgcccggatacccaaaccatcatcaaagtgaacagcgatttccactcattcgtgctgcccaggataggcagtaacacattggagatcgggctgagaacaagaatcaggaaaatgttagaggagcacaaggagccgtcacctctcattaccgccgaggacgtacaagaagctaagtgcgcagccgatgaggctaaggaggtgcgtgaagccgaggagttgcgcgcagctctaccacctttggcagctgatgttgaggagcccactctggaagccgatgtcgacttgatgttacaagaggctggggccggctcagtggagacacctcgtggcttgataaaggttaccagctacgctggcgaggacaagatcggctcttacgctgtgctttctccgcaggctgtactcaagagtgaaaaattatcttgcatccaccctctcgctgaacaagtcatagtgataacacactctggccgaaaagggcgttatgccgtggaaccataccatggtaaagtagtggtgccagagggacatgcaatacccgtccaggactttcaagctctgagtgaaagtgccaccattgtgtacaacgaacgtgagttcgtaaacaggtacctgcaccatattgccacacatggaggagcgctgaacactgatgaagaatattacaaaactgtcaagcccagcgagcacgacggcgaatacctgtacgacatcgacaggaaacagtgcgtcaagaaagagctagtcactgggctagggctcacaggcgagctggtcgatcctcccttccatgaattcgcctacgagagtctgagaacacgaccagccgctccttaccaagtaccaaccataggggtgtatggcgtgccaggatcaggcaagtctggcatcattaaaagcgcagtcaccaaaaaagatctagtggtgagcgccaagaaagaaaactgtgcagaaattataagggacgtcaagaaaatgaaagggctggacgtcaatgccagaactgtggactcagtgctcttgaatggatgcaaacaccccgtagagaccctgtatattgacgaggcttttgcttgtcatgcaggtactctcagagcgctcatagccattataagacctaaaaaggcagtgctctgcggagatcccaaacagtgcggtttttttaacatgatgtgcctgaaagtgcattttaaccacgagatttgcacacaagtcttccacaaaagcatctctcgccgttgcactaaatctgtgacttcggtcgtctcaaccttgttttacgacaaaaaaatgagaacgacgaatccgaaagagactaagattgtgattgacactaccggcagtaccaaacctaagcaggacgatctcattctcacttgtttcagagggtgggtgaagcagttgcaaatagattacaaaggcaacgaaataatgacggcagctgcctctcaagggctgacccgtaaaggtgtgtatgccgttcggtacaaggtgaatgaaaatcctctgtacgcacccacctcagaacatgtgaacgtcctactgacccgcacggaggaccgcatcgtgtggaaaacactagccggcgacccatggataaaaacactgactgccaagtaccctgggaatttcactgccacgatagaggagtggcaagcagagcatgatgccatcatgaggcacatcttggagagaccggaccctaccgacgtcttccagaataaggcaaacgtgtgttgggccaaggctttagtgccggtgctgaagaccgctggcatagacatgaccactgaacaatggaacactgtggattattttgaaacggacaaagctcactcagcagagatagtattgaaccaactatgcgtgaggttctttggactcgatctggactccggtctattttctgcacccactgttccgttatccattaggaataatcactgggataactccccgtcgcctaacatgtacgggctgaataaagaagtggtccgtcagctctctcgcaggtacccacaactgcctcgggcagttgccactggtagagtctatgacatgaacactggtacactgcgcaattatgatccgcgcataaacctagtacctgtaaacagaagactgcctcatgctttagtcctccaccataatgaacacccacagagtgacttttcttcattcgtcagcaaattgaagggcagaactgtcctggtggtcggggaaaagttgtccgtcccaggcaaaatggttgactggttgtcagaccggcctgaggctaccttcagagctcggctggatttaggcatcccaggtgatgtgcccaaatatgacataatatttgttaatgtgaggaccccatataaataccatcactatcagcagtgtgaagaccatgccattaagctaagcatgttgaccaagaaagcatgtctgcatctgaatcccggcggaacctgtgtcagcataggttatggttacgctgacagggccagcgaaagcatcattggtgctatagcgcggcagttcaagttttcccgagtatgcaaaccgaaatcctcacttgaggagacggaagttctgtttgtattcattgggtacgatcgcaaggcccgtacgcacaatccttacaagctatcatcaaccttgaccaacatttatacaggttccagactccacgaagccggatgtgcaccctcatatcatgtggtgcgaggggatattgccacggccaccgaaggagtgattataaatgctgctaacagcaaaggacaacctggcggaggggtgtgcggagcgctgtataagaaattcccggaaagtttcgatttacagccgatcgaagtaggaaaagcgcgactggtcaaaggtgcagctaaacatatcattcatgccgtaggaccaaacttcaacaaagtttcggaggttgaaggtgacaaacagttggcagaggcttatgagtccatcgctaagattgtcaacgataacaattacaagtcagtagcgattccactgttgtccaccggcatcttttccgggaacaaagatcgactaacccaatcattgaaccatttgctgacagctttagacaccactgatgcagatgtagccatatactgcagggacaagaaatgggaaatgactctcaaggaagcagtggctaggagagaagcagtggaggagatatgcatatccgacgattcttcagtgacagaacctgatgcagagctggtgagggtgcatcccaagagttctttggctggaaggaagggctacagcacaagcgatggcaaaactttctcatatttggaagggaccaagtttcaccaggcggccaaggatatagcagaaattaatgccatgtggcccgttgcaacggaggccaatgagcaggtatgcatgtatatcctcggagaaagcatgagcagtattaggtcgaaatgccccgtcgaggagtcggaagcctccacaccacctagcacgctgccttgcttgtgcatccatgccatgactccagaaagagtacagcgcctaaaagcctcacgtccagaacaaattactgtgtgctcatcctttccattgccgaagtatagaatcactggtgtgcagaagatccaatgctcccagcctatattgttctcaccgaaagtgcctgcgtatattcatccaaggaagtatctcgtggaaacaccaccggtagacgagactccggagccatcggcagagaaccaatccacagaggggacacctgaacaaccaccacttataaccgaggatgagaccaggactagaacgcctgagccgatcatcatcgaagaagaagaagaagatagcataagtttgctgtcagatggcccgacccaccaggtgctgcaagtcgaggcagacattcacgggccgccctctgtatctagctcatcctggtccattcctcatgcatccgactttgatgtggacagtttatccatacttgacaccctggagggagctagcgtgaccagcggggcaacgtcagccgagactaactcttacttcgcaaagagtatggagtttctggcgcgaccggtgcctgcgcctcgaacagtattcaggaaccctccacatcccgctccgcgcacaagaacaccgtcacttgcacccagcagggcctgctccagaaccagcctagtttccaccccgccaggcgtgaatagggtgatcactagagaggagctcgaagcgcttaccccgtcacgcactcctagcaggtcggtctccagaaccagcctggtctccaacccgccaggcgtaaatagggtgattacaagagaggagtttgaggcgttcgtagcacaacaacaatgacggtttgatgcgggtgcatacatcttttcctccgacaccggtcaagggcatttacaacaaaaatcagtaaggcaaacggtgctatccgaagtggtgttggagaggaccgaattggagatttcgtatgccccgcgcctcgaccaagaaaaagaagaattactacgcaagaaattacagttaaatcccacacctgctaacagaagcagataccagtccaggaaggtggagaacatgaaagccataacagctagacgtattctgcaaggcctagggcattatttgaaggcagaaggaaaagtggagtgctaccgaaccctgcatcctgttcctttgtattcatctagtgtgaaccgtgccttttcaagccccaaggtcgcagtggaagcctgtaacgccatgttgaaagagaactttccgactgtggcttcttactgtattattccagagtacgatgcctatttggacatggttgacggagcttcatgctgcttagacactgccagtttttgccctgcaaagctgcgcagctttccaaagaaacactcctatttggaacccacaatacgatcggcagtgccttcagcgatccagaacacgctccagaacgtcctggcagctgccacaaaaagaaattgcaatgtcacgcaaatgagagaattgcccgtattggattcggcggcctttaatgtggaatgcttcaagaaatatgcgtgtaataatgaatattgggaaacgtttaaagaaaaccccatcaggcttactgaagaaaacgtggtaaattacattaccaaattaaaaggaccaaaagctgctgctctttttgcgaagacacataatttgaatatgttgcaggacataccaatggacaggtttgtaatggacttaaagagagacgtgaaagtgactccaggaacaaaacatactgaagaacggcccaaggtacaggtgatccaggctgccgatccgctagcaacagcgtatctgtgcggaatccaccgagagctggttaggagattaaatgcggtcctgcttccgaacattcatacactgtttgatatgtcggctgaagactttgacgctattatagccgagcacttccagcctggggattgtgttctggaaactgacatcgcgtcgtttgataaaagtgaggacgacgccatggctctgaccgcgttaatgattctggaagacttaggtgtggacgcagagctgttgacgctgattgaggcggctttcggcgaaatttcatcaatacatttgcccactaaaactaaatttaaattcggagccatgatgaaatctggaatgttcctcacactgtttgtgaacacagtcattaacattgtaatcgcaagcagagtgttgagagaacggctaaccggatcaccatgtgcagcattcattggagatgacaatatcgtgaaaggagtcaaatcggacaaattaatggcagacaggtgcgccacctggttgaatatggaagtcaagattatagatgctgtggtgggcgagaaagcgccttatttctgtggagggtttattttgtgtgactccgtgaccggcacagcgtgccgtgtggcagaccccctaaaaaggctgtttaagctaggcaaacctctggcagcagacgatgaacatgatgatgacaggagaagggcattgcatgaggagtcaacacgctggaaccgagtgggtattctttcagagctgtgcaaggcagtagaatcaaggtatgaaaccgtaggaacttccatcatagttatggccatgactactctagctagcagtgttaaatcattcagctacctgagaggggcccctataactctctacggctaacctgaatggactacgacatagtctagtccgccaagactagtatgttcgtgttcctggtgctgctgcctctggtgtccagccagtgtgtgaacctgaccaccagaacacagctgcctccagcctacaccaacagctttaccagaggcgtgtactaccccgacaaggtgttcagatccagcgtgctgcactctacccaggacctgttcctgcctttcttcagcaacgtgacctggttccacgccatccacgtgtccggcaccaatggcaccaagagattcgacaaccccgtgctgcccttcaacgacggggtgtactttgccagcaccgagaagtccaacatcatcagaggctggatcttcggcaccacactggacagcaagacccagagcctgctgatcgtgaacaacgccaccaacgtggtcatcaaagtgtgcgagttccagttctgcaacgaccccttcctgggcgtctactaccacaagaacaacaagagctggatggaaagcgagttccgggtgtacagcagcgccaacaactgcaccttcgagtacgtgtcccagcctttcctgatggacctggaaggcaagcagggcaacttcaagaacctgcgcgagttcgtgtttaagaacatcgacggctacttcaagatctacagcaagcacacccctatcaacctcgtgcgggatctgcctcagggcttctctgctctggaacccctggtggatctgcccatcggcatcaacatcacccggtttcagacactgctggccctgcacagaagctacctgacacctggcgatagcagcagcggatggacagctggtgccgccgcttactatgtgggctacctgcagcctagaaccttcctgctgaagtacaacgagaacggcaccatcaccgacgccgtggattgtgctctggatcctctgagcgagacaaagtgcaccctgaagtccttcaccgtggaaaagggcatctaccagaccagcaacttccgggtgcagcccaccgaatccatcgtgcggttccccaatatcaccaatctgtgccccttcggcgaggtgttcaatgccaccagattcgcctctgtgtacgcctggaaccggaagcggatcagcaattgcgtggccgactactccgtgctgtacaactccgccagcttcagcaccttcaagtgctacggcgtgtcccctaccaagctgaacgacctgtgcttcacaaacgtgtacgccgacagcttcgtgatccggggagatgaagtgcggcagattgcccctggacagacaggcaagatcgccgactacaactacaagctgcccgacgacttcaccggctgtgtgattgcctggaacagcaacaacctggactccaaagtcggcggcaactacaattacctgtaccggctgttccggaagtccaatctgaagcccttcgagcgggacatctccaccgagatctatcaggccggcagcaccccttgtaacggcgtggaaggcttcaactgctacttcccactgcagtcctacggctttcagcccacaaatggcgtgggctatcagccctacagagtggtggtgctgagcttcgaactgctgcatgcccctgccacagtgtgcggccctaagaaaagcaccaatctcgtgaagaacaaatgcgtgaacttcaacttcaacggcctgaccggcaccggcgtgctgacagagagcaacaagaagttcctgccattccagcagtttggccgggatatcgccgataccacagacgccgttagagatccccagacactggaaatcctggacatcaccccttgcagcttcggcggagtgtctgtgatcacccctggcaccaacaccagcaatcaggtggcagtgctgtaccaggacgtgaactgtaccgaagtgcccgtggccattcacgccgatcagctgacacctacatggcgggtgtactccaccggcagcaatgtgtttcagaccagagccggctgtctgatcggagccgagcacgtgaacaatagctacgagtgcgacatccccatcggcgctggaatctgcgccagctaccagacacagacaaacagccctcggagagccagaagcgtggccagccagagcatcattgcctacacaatgtctctgggcgccgagaacagcgtggcctactccaacaactctatcgctatccccaccaacttcaccatcagcgtgaccacagagatcctgcctgtgtccatgaccaagaccagcgtggactgcaccatgtacatctgcggcgattccaccgagtgctccaacctgctgctgcagtacggcagcttctgcacccagctgaatagagccctgacagggatcgccgtggaacaggacaagaacacccaagaggtgttcgcccaagtgaagcagatctacaagacccctcctatcaaggacttcggcggcttcaatttcagccagattctgcccgatcctagcaagcccagcaagcggagcttcatcgaggacctgctgttcaacaaagtgacactggccgacgccggcttcatcaagcagtatggcgattgtctgggcgacattgccgccagggatctgatttgcgcccagaagtttaacggactgacagtgctgcctcctctgctgaccgatgagatgatcgcccagtacacatctgccctgctggccggcacaatcacaagcggctggacatttggagcaggcgccgctctgcagatcccctttgctatgcagatggcctaccggttcaacggcatcggagtgacccagaatgtgctgtacgagaaccagaagctgatcgccaaccagttcaacagcgccatcggcaagatccaggacagcctgagcagcacagcaagcgccctgggaaagctgcaggacgtggtcaaccagaatgcccaggcactgaacaccctggtcaagcagctgtcctccaacttcggcgccatcagctctgtgctgaacgatatcctgagcagactggaccctcctgaggccgaggtgcagatcgacagactgatcacaggcagactgcagagcctccagacatacgtgacccagcagctgatcagagccgccgagattagagcctctgccaatctggccgccaccaagatgtctgagtgtgtgctgggccagagcaagagagtggacttttgcggcaagggctaccacctgatgagcttccctcagtctgcccctcacggcgtggtgtttctgcacgtgacatatgtgcccgctcaagagaagaatttcaccaccgctccagccatctgccacgacggcaaagcccactttcctagagaaggcgtgttcgtgtccaacggcacccattggttcgtgacacagcggaacttctacgagccccagatcatcaccaccgacaacaccttcgtgtctggcaactgcgacgtcgtgatcggcattgtgaacaataccgtgtacgaccctctgcagcccgagctggacagcttcaaagaggaactggacaagtactttaagaaccacacaagccccgacgtggacctgggcgatatcagcggaatcaatgccagcgtcgtgaacatccagaaagagatcgaccggctgaacgaggtggccaagaatctgaacgagagcctgatcgacctgcaagaactggggaagtacgagcagtacatcaagtggccctggtacatctggctgggctttatcgccggactgattgccatcgtgatggtcacaatcatgctgtgttgcatgaccagctgctgtagctgcctgaagggctgttgtagctgtggcagctgctgcaagttcgacgaggacgattctgagcccgtgctgaagggcgtgaaactgcactacacatgatgactcgagctggtactgcatgcacgcaatgctagctgcccctttcccgtcctgggtaccccgagtctcccccgacctcgggtcccaggtatgctcccacctccacctgccccactcaccacctctgctagttccagacacctcccaagcacgcagcaatgcagctcaaaacgcttagcctagccacacccccacgggaaacagcagtgattaacctttagcaataaacgaaagtttaactaagctatactaaccccagggttggtcaatttcgtgccagccacaccgcggccgcatgaatacagcagcaattggcaagctgcttacatagaactcgcggcgattggcatgccgccttaaaatttttattttattttttcttttcttttccgaatcggattttgtttttaatatttcaaaaaaaaaaaaaaaaaaaaaaaaaaaaaagcatatgactaaaaaaaaaaaaaaaaaaaaaaaaaaaaaaaaaaaaaaaaaaaaaaaaaaaaaaaaaaaaaaaaaaaaaa

SEQ ID NO: 35 - RNA, 8896 nt, synthetic construct
  source 1..8896: mol_type = other RNA
gatgggcggcgcatgagagaagcccagaccaattacctacccaaaatggagaaagttcacgttgacatcgaggaagacagcccattcctcagagctttgcagcggagcttcccgcagtttgaggtagaagccaagcaggtcactgataatgaccatgctaatgccagagcgttttcgcatctggcttcaaaactgatcgaaacggaggtggacccatccgacacgatccttgacattggaagtgcgcccgcccgcagaatgtattctaagcacaagtatcattgtatctgtccgatgagatgtgcggaagatccggacagattgtataagtatgcaactaagctgaagaaaaactgtaaggaaataactgataaggaattggacaagaaaatgaaggagctcgccgccgtcatgagcgaccctgacctggaaactgagactatgtgcctccacgacgacgagtcgtgtcgctacgaagggcaagtcgctgtttaccaggatgtatacgcggttgacggaccgacaagtctctatcaccaagccaataagggagttagagtcgcctactggataggctttgacaccaccccttttatgtttaagaacttggctggagcatatccatcatactctaccaactgggccgacgaaaccgtgttaacggctcgtaacataggcctatgcagctctgacgttatggagcggtcacgtagagggatgtccattcttagaaagaagtatttgaaaccatccaacaatgttctattctctgttggctcgaccatctaccacgaaaagagggacttactgaggagctggcacctgccgtctgtatttcacttacgtggcaagcaaaattacacatgtcggtgtgagactatagttagttgcgacgggtacgtcgttaaaagaatagctatcagtccaggcctgtatgggaagccttcaggctatgctgctacgatgcaccgcgagggattcttgtgctgcaaagtgacagacacattgaacggggagagggtctcttttcccgtgtgcacgtatgtgccagctacattgtgtgaccaaatgactggcatactggcaacagatgtcagtgcggacgacgcgcaaaaactgctggttgggctcaaccagcgtatagtcgtcaacggtcgcacccagagaaacaccaataccatgaaaaattaccttttgcccgtagtggcccaggcatttgctaggtgggcaaaggaatataaggaagatcaagaagatgaaaggccactaggactacgagatagacagttagtcatggggtgttgttgggcttttagaaggcacaagataacatctatttataagcgcccggatacccaaaccatcatcaaagtgaacagcgatttccactcattcgtgctgcccaggataggcagtaacacattggagatcgggctgagaacaagaatcaggaaaatgttagaggagcacaaggagccgtcacctctcattaccgccgaggacgtacaagaagctaagtgcgcagccgatgaggctaaggaggtgcgtgaagccgaggagttgcgcgcagctctaccacctttggcagctgatgttgaggagcccactctggaagccgatgtcgacttgatgttacaagaggctggggccggctcagtggagacacctcgtggcttgataaaggttaccagctacgctggcgaggacaagatcggctcttacgctgtgctttctccgcaggctgtactcaagagtgaaaaattatcttgcatccaccctctcgctgaacaagtcatagtgataacacactctggccgaaaagggcgttatgccgtggaaccataccatggtaaagtagtggtgccagagggacatgcaatacccgtccaggactttcaagctctgagtgaaagtgccaccattgtgtacaacgaacgtgagttcgtaaacaggtacctgcaccatattgccacacatggaggagcgctgaacactgatgaagaatattacaaaactgtcaagcccagcgagcacgacggcgaatacctgtacgacatcgacaggaaacagtgcgtcaagaaagagctagtcactgggctagggctcacaggcgagctggtcgatcctcccttccatgaattcgcctacgagagtctgagaacacgaccagccgctccttaccaagtaccaaccataggggtgtatggcgtgccaggatcaggcaagtctggcatcattaaaagcgcagtcaccaaaaaagatctagtggtgagcgccaagaaagaaaactgtgcagaaattataagggacgtcaagaaaatgaaagggctggacgtcaatgccagaactgtggactcagtgctcttgaatggatgcaaacaccccgtagagaccctgtatattgacgaggcttttgcttgtcatgcaggtactctcagagcgctcatagccattataagacctaaaaaggcagtgctctgcggagatcccaaacagtgcggtttttttaacatgatgtgcctgaaagtgcattttaaccacgagatttgcacacaagtcttccacaaaagcatctctcgccgttgcactaaatctgtgacttcggtcgtctcaaccttgttttacgacaaaaaaatgagaacgacgaatccgaaagagactaagattgtgattgacactaccggcagtaccaaacctaagcaggacgatctcattctcacttgtttcagagggtgggtgaagcagttgcaaatagattacaaaggcaacgaaataatgacggcagctgcctctcaagggctgacccgtaaaggtgtgtatgccgttcggtacaaggtgaatgaaaatcctctgtacgcacccacctcagaacatgtgaacgtcctactgacccgcacggaggaccgcatcgtgtggaaaacactagccggcgacccatggataaaaacactgactgccaagtaccctgggaatttcactgccacgatagaggagtggcaagcagagcatgatgccatcatgaggcacatcttggagagaccggaccctaccgacgtcttccagaataaggcaaacgtgtgttgggccaaggctttagtgccggtgctgaagaccgctggcatagacatgaccactgaacaatggaacactgtggattattttgaaacggacaaagctcactcagcagagatagtattgaaccaactatgcgtgaggttctttggactcgatctggactccggtctattttctgcacccactgttccgttatccattaggaataatcactgggataactccccgtcgcctaacatgtacgggctgaataaagaagtggtccgtcagctctctcgcaggtacccacaactgcctcgggcagttgccactggtagagtctatgacatgaacactggtacactgcgcaattatgatccgcgcataaacctagtacctgtaaacagaagactgcctcatgctttagtcctccaccataatgaacacccacagagtgacttttcttcattcgtcagcaaattgaagggcagaactgtcctggtggtcggggaaaagttgtccgtcccaggcaaaatggttgactggttgtcagaccggcctgaggctaccttcagagctcggctggatttaggcatcccaggtgatgtgcccaaatatgacataatatttgttaatgtgaggaccccatataaataccatcactatcagcagtgtgaagaccatgccattaagctaagcatgttgaccaagaaagcatgtctgcatctgaatcccggcggaacctgtgtcagcataggttatggttacgctgacagggccagcgaaagcatcattggtgctatagcgcggcagttcaagttttcccgagtatgcaaaccgaaatcctcacttgaggagacggaagttctgtttgtattcattgggtacgatcgcaaggcccgtacgcacaatccttacaagctatcatcaaccttgaccaacatttatacaggttccagactccacgaagccggatgtgcaccctcatatcatgtggtgcgaggggatattgccacggccaccgaaggagtgattataaatgctgctaacagcaaaggacaacctggcggaggggtgtgcggagcgctgtataagaaattcccggaaagtttcgatttacagccgatcgaagtaggaaaagcgcgactggtcaaaggtgcagctaaacatatcattcatgccgtaggaccaaacttcaacaaagtttcggaggttgaaggtgacaaacagttggcagaggcttatgagtccatcgctaagattgtcaacgataacaattacaagtcagtagcgattccactgttgtccaccggcatcttttccgggaacaaagatcgactaacccaatcattgaaccatttgctgacagctttagacaccactgatgcagatgtagccatatactgcagggacaagaaatgggaaatgactctcaaggaagcagtggctaggagagaagcagtggaggagatatgcatatccgacgattcttcagtgacagaacctgatgcagagctggtgagggtgcatcccaagagttctttggctggaaggaagggctacagcacaagcgatggcaaaactttctcatatttggaagggaccaagtttcaccaggcggccaaggatatagcagaaattaatgccatgtggcccgttgcaacggaggccaatgagcaggtatgcatgtatatcctcggagaaagcatgagcagtattaggtcgaaatgccccgtcgaggagtcggaagcctccacaccacctagcacgctgccttgcttgtgcatccatgccatgactccagaaagagtacagcgcctaaaagcctcacgtccagaacaaattactgtgtgctcatcctttccattgccgaagtatagaatcactggtgtgcagaagatccaatgctcccagcctatattgttctcaccgaaagtgcctgcgtatattcatccaaggaagtatctcgtggaaacaccaccggtagacgagactccggagccatcggcagagaaccaatccacagaggggacacctgaacaaccaccacttataaccgaggatgagaccaggactagaacgcctgagccgatcatcatcgaagaagaagaagaagatagcataagtttgctgtcagatggcccgacccaccaggtgctgcaagtcgaggcagacattcacgggccgccctctgtatctagctcatcctggtccattcctcatgcatccgactttgatgtggacagtttatccatacttgacaccctggagggagctagcgtgaccagcggggcaacgtcagccgagactaactcttacttcgcaaagagtatggagtttctggcgcgaccggtgcctgcgcctcgaacagtattcaggaaccctccacatcccgctccgcgcacaagaacaccgtcacttgcacccagcagggcctgctccagaaccagcctagtttccaccccgccaggcgtgaatagggtgatcactagagaggagctcgaagcgcttaccccgtcacgcactcctagcaggtcggtctccagaaccagcctggtctccaacccgccaggcgtaaatagggtgattacaagagaggagtttgaggcgttcgtagcacaacaacaatgacggtttgatgcgggtgcatacatcttttcctccgacaccggtcaagggcatttacaacaaaaatcagtaaggcaaacggtgctatccgaagtggtgttggagaggaccgaattggagatttcgtatgccccgcgcctcgaccaagaaaaagaagaattactacgcaagaaattacagttaaatcccacacctgctaacagaagcagataccagtccaggaaggtggagaacatgaaagccataacagctagacgtattctgcaaggcctagggcattatttgaaggcagaaggaaaagtggagtgctaccgaaccctgcatcctgttcctttgtattcatctagtgtgaaccgtgccttttcaagccccaaggtcgcagtggaagcctgtaacgccatgttgaaagagaactttccgactgtggcttcttactgtattattccagagtacgatgcctatttggacatggttgacggagcttcatgctgcttagacactgccagtttttgccctgcaaagctgcgcagctttccaaagaaacactcctatttggaacccacaatacgatcggcagtgccttcagcgatccagaacacgctccagaacgtcctggcagctgccacaaaaagaaattgcaatgtcacgcaaatgagagaattgcccgtattggattcggcggcctttaatgtggaatgcttcaagaaatatgcgtgtaataatgaatattgggaaacgtttaaagaaaaccccatcaggcttactgaagaaaacgtggtaaattacattaccaaattaaaaggaccaaaagctgctgctctttttgcgaagacacataatttgaatatgttgcaggacataccaatggacaggtttgtaatggacttaaagagagacgtgaaagtgactccaggaacaaaacatactgaagaacggcccaaggtacaggtgatccaggctgccgatccgctagcaacagcgtatctgtgcggaatccaccgagagctggttaggagattaaatgcggtcctgcttccgaacattcatacactgtttgatatgtcggctgaagactttgacgctattatagccgagcacttccagcctggggattgtgttctggaaactgacatcgcgtcgtttgataaaagtgaggacgacgccatggctctgaccgcgttaatgattctggaagacttaggtgtggacgcagagctgttgacgctgattgaggcggctttcggcgaaatttcatcaatacatttgcccactaaaactaaatttaaattcggagccatgatgaaatctggaatgttcctcacactgtttgtgaacacagtcattaacattgtaatcgcaagcagagtgttgagagaacggctaaccggatcaccatgtgcagcattcattggagatgacaatatcgtgaaaggagtcaaatcggacaaattaatggcagacaggtgcgccacctggttgaatatggaagtcaagattatagatgctgtggtgggcgagaaagcgccttatttctgtggagggtttattttgtgtgactccgtgaccggcacagcgtgccgtgtggcagaccccctaaaaaggctgtttaagctaggcaaacctctggcagcagacgatgaacatgatgatgacaggagaagggcattgcatgaggagtcaacacgctggaaccgagtgggtattctttcagagctgtgcaaggcagtagaatcaaggtatgaaaccgtaggaacttccatcatagttatggccatgactactctagctagcagtgttaaatcattcagctacctgagaggggcccctataactctctacggctaacctgaatggactacgacatagtctagtccgccaagactagtatgtttgtgtttcttgtgctgctgcctcttgtgtcttctcagtgtgtggtgagatttccaaatattacaaatctgtgtccatttggagaagtgtttaatgcaacaagatttgcatctgtgtatgcatggaatagaaaaagaatttctaattgtgtggctgattattctgtgctgtataatagtgcttctttttccacatttaaatgttatggagtgtctccaacaaaattaaatgatttatgttttacaaatgtgtatgctgattcttttgtgatcagaggtgatgaagtgagacagattgcccccggacagacaggaaaaattgctgattacaattacaaactgcctgatgattttacaggatgtgtgattgcttggaattctaataatttagattctaaagtgggaggaaattacaattatctgtacagactgtttagaaaatcaaatctgaaaccttttgaaagagatatttcaacagaaatttatcaggctggatcaacaccttgtaatggagtggaaggatttaattgttattttccattacagagctatggatttcagccaaccaatggtgtgggatatcagccatatagagtggtggtgctgtcttttgaactgctgcatgcacctgcaacagtgtgtggacctaaaggctcccccggctccggctccggatctggttatattcctgaagctccaagagatgggcaagcttacgttcgtaaagatggcgaatgggtattactttctacctttttaggccggtccctggaggtgctgttccagggccccggctgatgactcgagctggtactgcatgcacgcaatgctagctgcccctttcccgtcctgggtaccccgagtctcccccgacctcgggtcccaggtatgctcccacctccacctgccccactcaccacctctgctagttccagacacctcccaagcacgcagcaatgcagctcaaaacgcttagcctagccacacccccacgggaaacagcagtgattaacctttagcaataaacgaaagtttaactaagctatactaaccccagggttggtcaatttcgtgccagccacaccgcggccgcatgaatacagcagcaattggcaagctgcttacatagaactcgcggcgattggcatgccgccttaaaatttttattttattttttcttttcttttccgaatcggattttgtttttaatatttcaaaaaaaaaaaaaaaaaaaaaaaaaaaaaagcatatgactaaaaaaaaaaaaaaaaaaaaaaaaaaaaaaaaaaaaaaaaaaaaaaaaaaaaaaaaaaaaaaaaaaaaaa

SEQ ID NO: 36 - RNA, 9079 nt, synthetic construct
  source 1..9079: mol_type = other RNA
gatgggcggcgcatgagagaagcccagaccaattacctacccaaaatggagaaagttcacgttgacatcgaggaagacagcccattcctcagagctttgcagcggagcttcccgcagtttgaggtagaagccaagcaggtcactgataatgaccatgctaatgccagagcgttttcgcatctggcttcaaaactgatcgaaacggaggtggacccatccgacacgatccttgacattggaagtgcgcccgcccgcagaatgtattctaagcacaagtatcattgtatctgtccgatgagatgtgcggaagatccggacagattgtataagtatgcaactaagctgaagaaaaactgtaaggaaataactgataaggaattggacaagaaaatgaaggagctcgccgccgtcatgagcgaccctgacctggaaactgagactatgtgcctccacgacgacgagtcgtgtcgctacgaagggcaagtcgctgtttaccaggatgtatacgcggttgacggaccgacaagtctctatcaccaagccaataagggagttagagtcgcctactggataggctttgacaccaccccttttatgtttaagaacttggctggagcatatccatcatactctaccaactgggccgacgaaaccgtgttaacggctcgtaacataggcctatgcagctctgacgttatggagcggtcacgtagagggatgtccattcttagaaagaagtatttgaaaccatccaacaatgttctattctctgttggctcgaccatctaccacgaaaagagggacttactgaggagctggcacctgccgtctgtatttcacttacgtggcaagcaaaattacacatgtcggtgtgagactatagttagttgcgacgggtacgtcgttaaaagaatagctatcagtccaggcctgtatgggaagccttcaggctatgctgctacgatgcaccgcgagggattcttgtgctgcaaagtgacagacacattgaacggggagagggtctcttttcccgtgtgcacgtatgtgccagctacattgtgtgaccaaatgactggcatactggcaacagatgtcagtgcggacgacgcgcaaaaactgctggttgggctcaaccagcgtatagtcgtcaacggtcgcacccagagaaacaccaataccatgaaaaattaccttttgcccgtagtggcccaggcatttgctaggtgggcaaaggaatataaggaagatcaagaagatgaaaggccactaggactacgagatagacagttagtcatggggtgttgttgggcttttagaaggcacaagataacatctatttataagcgcccggatacccaaaccatcatcaaagtgaacagcgatttccactcattcgtgctgcccaggataggcagtaacacattggagatcgggctgagaacaagaatcaggaaaatgttagaggagcacaaggagccgtcacctctcattaccgccgaggacgtacaagaagctaagtgcgcagccgatgaggctaaggaggtgcgtgaagccgaggagttgcgcgcagctctaccacctttggcagctgatgttgaggagcccactctggaagccgatgtcgacttgatgttacaagaggctggggccggctcagtggagacacctcgtggcttgataaaggttaccagctacgctggcgaggacaagatcggctcttacgctgtgctttctccgcaggctgtactcaagagtgaaaaattatcttgcatccaccctctcgctgaacaagtcatagtgataacacactctggccgaaaagggcgttatgccgtggaaccataccatggtaaagtagtggtgccagagggacatgcaatacccgtccaggactttcaagctctgagtgaaagtgccaccattgtgtacaacgaacgtgagttcgtaaacaggtacctgcaccatattgccacacatggaggagcgctgaacactgatgaagaatattacaaaactgtcaagcccagcgagcacgacggcgaatacctgtacgacatcgacaggaaacagtgcgtcaagaaagagctagtcactgggctagggctcacaggcgagctggtcgatcctcccttccatgaattcgcctacgagagtctgagaacacgaccagccgctccttaccaagtaccaaccataggggtgtatggcgtgccaggatcaggcaagtctggcatcattaaaagcgcagtcaccaaaaaagatctagtggtgagcgccaagaaagaaaactgtgcagaaattataagggacgtcaagaaaatgaaagggctggacgtcaatgccagaactgtggactcagtgctcttgaatggatgcaaacaccccgtagagaccctgtatattgacgaggcttttgcttgtcatgcaggtactctcagagcgctcatagccattataagacctaaaaaggcagtgctctgcggagatcccaaacagtgcggtttttttaacatgatgtgcctgaaagtgcattttaaccacgagatttgcacacaagtcttccacaaaagcatctctcgccgttgcactaaatctgtgacttcggtcgtctcaaccttgttttacgacaaaaaaatgagaacgacgaatccgaaagagactaagattgtgattgacactaccggcagtaccaaacctaagcaggacgatctcattctcacttgtttcagagggtgggtgaagcagttgcaaatagattacaaaggcaacgaaataatgacggcagctgcctctcaagggctgacccgtaaaggtgtgtatgccgttcggtacaaggtgaatgaaaatcctctgtacgcacccacctcagaacatgtgaacgtcctactgacccgcacggaggaccgcatcgtgtggaaaacactagccggcgacccatggataaaaacactgactgccaagtaccctgggaatttcactgccacgatagaggagtggcaagcagagcatgatgccatcatgaggcacatcttggagagaccggaccctaccgacgtcttccagaataaggcaaacgtgtgttgggccaaggctttagtgccggtgctgaagaccgctggcatagacatgaccactgaacaatggaacactgtggattattttgaaacggacaaagctcactcagcagagatagtattgaaccaactatgcgtgaggttctttggactcgatctggactccggtctattttctgcacccactgttccgttatccattaggaataatcactgggataactccccgtcgcctaacatgtacgggctgaataaagaagtggtccgtcagctctctcgcaggtacccacaactgcctcgggcagttgccactggtagagtctatgacatgaacactggtacactgcgcaattatgatccgcgcataaacctagtacctgtaaacagaagactgcctcatgctttagtcctccaccataatgaacacccacagagtgacttttcttcattcgtcagcaaattgaagggcagaactgtcctggtggtcggggaaaagttgtccgtcccaggcaaaatggttgactggttgtcagaccggcctgaggctaccttcagagctcggctggatttaggcatcccaggtgatgtgcccaaatatgacataatatttgttaatgtgaggaccccatataaataccatcactatcagcagtgtgaagaccatgccattaagctaagcatgttgaccaagaaagcatgtctgcatctgaatcccggcggaacctgtgtcagcataggttatggttacgctgacagggccagcgaaagcatcattggtgctatagcgcggcagttcaagttttcccgagtatgcaaaccgaaatcctcacttgaggagacggaagttctgtttgtattcattgggtacgatcgcaaggcccgtacgcacaatccttacaagctatcatcaaccttgaccaacatttatacaggttccagactccacgaagccggatgtgcaccctcatatcatgtggtgcgaggggatattgccacggccaccgaaggagtgattataaatgctgctaacagcaaaggacaacctggcggaggggtgtgcggagcgctgtataagaaattcccggaaagtttcgatttacagccgatcgaagtaggaaaagcgcgactggtcaaaggtgcagctaaacatatcattcatgccgtaggaccaaacttcaacaaagtttcggaggttgaaggtgacaaacagttggcagaggcttatgagtccatcgctaagattgtcaacgataacaattacaagtcagtagcgattccactgttgtccaccggcatcttttccgggaacaaagatcgactaacccaatcattgaaccatttgctgacagctttagacaccactgatgcagatgtagccatatactgcagggacaagaaatgggaaatgactctcaaggaagcagtggctaggagagaagcagtggaggagatatgcatatccgacgattcttcagtgacagaacctgatgcagagctggtgagggtgcatcccaagagttctttggctggaaggaagggctacagcacaagcgatggcaaaactttctcatatttggaagggaccaagtttcaccaggcggccaaggatatagcagaaattaatgccatgtggcccgttgcaacggaggccaatgagcaggtatgcatgtatatcctcggagaaagcatgagcagtattaggtcgaaatgccccgtcgaggagtcggaagcctccacaccacctagcacgctgccttgcttgtgcatccatgccatgactccagaaagagtacagcgcctaaaagcctcacgtccagaacaaattactgtgtgctcatcctttccattgccgaagtatagaatcactggtgtgcagaagatccaatgctcccagcctatattgttctcaccgaaagtgcctgcgtatattcatccaaggaagtatctcgtggaaacaccaccggtagacgagactccggagccatcggcagagaaccaatccacagaggggacacctgaacaaccaccacttataaccgaggatgagaccaggactagaacgcctgagccgatcatcatcgaagaagaagaagaagatagcataagtttgctgtcagatggcccgacccaccaggtgctgcaagtcgaggcagacattcacgggccgccctctgtatctagctcatcctggtccattcctcatgcatccgactttgatgtggacagtttatccatacttgacaccctggagggagctagcgtgaccagcggggcaacgtcagccgagactaactcttacttcgcaaagagtatggagtttctggcgcgaccggtgcctgcgcctcgaacagtattcaggaaccctccacatcccgctccgcgcacaagaacaccgtcacttgcacccagcagggcctgctccagaaccagcctagtttccaccccgccaggcgtgaatagggtgatcactagagaggagctcgaagcgcttaccccgtcacgcactcctagcaggtcggtctccagaaccagcctggtctccaacccgccaggcgtaaatagggtgattacaagagaggagtttgaggcgttcgtagcacaacaacaatgacggtttgatgcgggtgcatacatcttttcctccgacaccggtcaagggcatttacaacaaaaatcagtaaggcaaacggtgctatccgaagtggtgttggagaggaccgaattggagatttcgtatgccccgcgcctcgaccaagaaaaagaagaattactacgcaagaaattacagttaaatcccacacctgctaacagaagcagataccagtccaggaaggtggagaacatgaaagccataacagctagacgtattctgcaaggcctagggcattatttgaaggcagaaggaaaagtggagtgctaccgaaccctgcatcctgttcctttgtattcatctagtgtgaaccgtgccttttcaagccccaaggtcgcagtggaagcctgtaacgccatgttgaaagagaactttccgactgtggcttcttactgtattattccagagtacgatgcctatttggacatggttgacggagcttcatgctgcttagacactgccagtttttgccctgcaaagctgcgcagctttccaaagaaacactcctatttggaacccacaatacgatcggcagtgccttcagcgatccagaacacgctccagaacgtcctggcagctgccacaaaaagaaattgcaatgtcacgcaaatgagagaattgcccgtattggattcggcggcctttaatgtggaatgcttcaagaaatatgcgtgtaataatgaatattgggaaacgtttaaagaaaaccccatcaggcttactgaagaaaacgtggtaaattacattaccaaattaaaaggaccaaaagctgctgctctttttgcgaagacacataatttgaatatgttgcaggacataccaatggacaggtttgtaatggacttaaagagagacgtgaaagtgactccaggaacaaaacatactgaagaacggcccaaggtacaggtgatccaggctgccgatccgctagcaacagcgtatctgtgcggaatccaccgagagctggttaggagattaaatgcggtcctgcttccgaacattcatacactgtttgatatgtcggctgaagactttgacgctattatagccgagcacttccagcctggggattgtgttctggaaactgacatcgcgtcgtttgataaaagtgaggacgacgccatggctctgaccgcgttaatgattctggaagacttaggtgtggacgcagagctgttgacgctgattgaggcggctttcggcgaaatttcatcaatacatttgcccactaaaactaaatttaaattcggagccatgatgaaatctggaatgttcctcacactgtttgtgaacacagtcattaacattgtaatcgcaagcagagtgttgagagaacggctaaccggatcaccatgtgcagcattcattggagatgacaatatcgtgaaaggagtcaaatcggacaaattaatggcagacaggtgcgccacctggttgaatatggaagtcaagattatagatgctgtggtgggcgagaaagcgccttatttctgtggagggtttattttgtgtgactccgtgaccggcacagcgtgccgtgtggcagaccccctaaaaaggctgtttaagctaggcaaacctctggcagcagacgatgaacatgatgatgacaggagaagggcattgcatgaggagtcaacacgctggaaccgagtgggtattctttcagagctgtgcaaggcagtagaatcaaggtatgaaaccgtaggaacttccatcatagttatggccatgactactctagctagcagtgttaaatcattcagctacctgagaggggcccctataactctctacggctaacctgaatggactacgacatagtctagtccgccaagactagtatgtttgtgtttcttgtgctgctgcctcttgtgtcttctcagtgtgtggtgagatttccaaatattacaaatctgtgtccatttggagaagtgtttaatgcaacaagatttgcatctgtgtatgcatggaatagaaaaagaatttctaattgtgtggctgattattctgtgctgtataatagtgcttctttttccacatttaaatgttatggagtgtctccaacaaaattaaatgatttatgttttacaaatgtgtatgctgattcttttgtgatcagaggtgatgaagtgagacagattgcccccggacagacaggaaaaattgctgattacaattacaaactgcctgatgattttacaggatgtgtgattgcttggaattctaataatttagattctaaagtgggaggaaattacaattatctgtacagactgtttagaaaatcaaatctgaaaccttttgaaagagatatttcaacagaaatttatcaggctggatcaacaccttgtaatggagtggaaggatttaattgttattttccattacagagctatggatttcagccaaccaatggtgtgggatatcagccatatagagtggtggtgctgtcttttgaactgctgcatgcacctgcaacagtgtgtggacctaaaggctcccccggctccggctccggatctggttatattcctgaagctccaagagatgggcaagcttacgttcgtaaagatggcgaatgggtattactttctacctttttaggaagcggcagcggatctgaacagtacattaaatggccttggtacatttggcttggatttattgcaggattaattgcaattgtgatggtgacaattatgttatgttgtatgacatcatgttgttcttgtttaaaaggatgttgttcttgtggaagctgttgtaaatttgatgaagatgattctgaacctgtgttaaaaggagtgaaattgcattacacatgatgactcgagctggtactgcatgcacgcaatgctagctgcccctttcccgtcctgggtaccccgagtctcccccgacctcgggtcccaggtatgctcccacctccacctgccccactcaccacctctgctagttccagacacctcccaagcacgcagcaatgcagctcaaaacgcttagcctagccacacccccacgggaaacagcagtgattaacctttagcaataaacgaaagtttaactaagctatactaaccccagggttggtcaatttcgtgccagccacaccgcggccgcatgaatacagcagcaattggcaagctgcttacatagaactcgcggcgattggcatgccgccttaaaatttttattttattttttcttttcttttccgaatcggattttgtttttaatatttcaaaaaaaaaaaaaaaaaaaaaaaaaaaaaagcatatgactaaaaaaaaaaaaaaaaaaaaaaaaaaaaaaaaaaaaaaaaaaaaaaaaaaaaaaaaaaaaaaaaaaaaaa

SEQ ID NO: 37 - protein, 327 aa, synthetic construct
MFVFLVLLPLVSSQCVVRFPNITNLCPFGEVFNATRFASVYAWNRKRISNCVADYSVLYNSASFSTFKCYGVSPTKLNDLCFTNVYADSFVIRGDEVRQIAPGQTGKIADYNYKLPDDFTGCVIAWNSNNLDSKVGGNYNYLYRLFRKSNLKPFERDISTEIYQAGSTPCNGVEGFNCYFPLQSYGFQPTNGVGYQPYRVVVLSFELLHAPATVCGPKGSPGSGSGSGYIPEAPRDGQAYVRKDGEWVLLSTFLGSGSGSEQYIKWPWYIWLGFIAGLIAIVMVTIMLCCMTSCCSCLKGCCSCGSCCKFDEDDSEPVLKGVKLHYT

SEQ ID NO: 38 - protein, 311 aa, synthetic construct
MFVFLVLLPLVSSQCVNLTVRFPNITNLCPFGEVFNATRFASVYAWNRKRISNCVADYSVLYNSASFSTFKCYGVSPTKLNDLCFTNVYADSFVIRGDEVRQIAPGQTGKIADYNYKLPDDFTGCVIAWNSNNLDSKVGGNYNYLYRLFRKSNLKPFERDISTEIYQAGSTPCNGVEGFNCYFPLQSYGFQPTNGVGYQPYRVVVLSFELLHAPATVCGPKGSPGSGSGSGYIPEAPRDGQAYVRKDGEWVLLSTFLGSGSGSEQYIKWPWYIWLGFIAGLIAIVMVTIMLCCMTSCCSCLKGCCSCGSCC

SEQ ID NO: 39 - RNA, 1397 nt, synthetic construct
  source 1..1397: mol_type = other RNA
agaataaactagtattcttctggtccccacagactcagagagaacccgccaccatgtttgtgtttcttgtgctgctgcctcttgtgtcttctcagtgtgtgaatttgacagtgagatttccaaatattacaaatctgtgtccatttggagaagtgtttaatgcaacaagatttgcatctgtgtatgcatggaatagaaaaagaatttctaattgtgtggctgattattctgtgctgtataatagtgcttctttttccacatttaaatgttatggagtgtctccaacaaaattaaatgatttatgttttacaaatgtgtatgctgattcttttgtgatcagaggtgatgaagtgagacagattgcccccggacagacaggaaaaattgctgattacaattacaaactgcctgatgattttacaggatgtgtgattgcttggaattctaataatttagattctaaagtgggaggaaattacaattatctgtacagactgtttagaaaatcaaatctgaaaccttttgaaagagatatttcaacagaaatttatcaggctggatcaacaccttgtaatggagtggaaggatttaattgttattttccattacagagctatggatttcagccaaccaatggtgtgggatatcagccatatagagtggtggtgctgtcttttgaactgctgcatgcacctgcaacagtgtgtggacctaaaggctcccccggctccggctccggatctggttatattcctgaagctccaagagatgggcaagcttacgttcgtaaagatggcgaatgggtattactttctacctttttaggaagcggcagcggatctgaacagtacattaaatggccttggtacatttggcttggatttattgcaggattaattgcaattgtgatggtgacaattatgttatgttgtatgacatcatgttgttcttgtttaaaaggatgttgttcttgtggaagctgttgttgatgactcgagctggtactgcatgcacgcaatgctagctgcccctttcccgtcctgggtaccccgagtctcccccgacctcgggtcccaggtatgctcccacctccacctgccccactcaccacctctgctagttccagacacctcccaagcacgcagcaatgcagctcaaaacgcttagcctagccacacccccacgggaaacagcagtgattaacctttagcaataaacgaaagtttaactaagctatactaaccccagggttggtcaatttcgtgccagccacaccctggagctagcaaaaaaaaaaaaaaaaaaaaaaaaaaaaaagcatatgactaaaaaaaaaaaaaaaaaaaaaaaaaaaaaaaaaaaaaaaaaaaaaaaaaaaaaaaaaaaaaaaaaaaaaa

SEQ ID NO: 40 - protein, 314 aa, synthetic construct
  REGION 1..314: note = BNT162b3d
MDWIWRILFLVGAATGAHSQMQVRFPNITNLCPFGEVFNATRFASVYAWNRKRISNCVADYSVLYNSASFSTFKCYGVSPTKLNDLCFTNVYADSFVIRGDEVRQIAPGQTGKIADYNYKLPDDFTGCVIAWNSNNLDSKVGGNYNYLYRLFRKSNLKPFERDISTEIYQAGSTPCNGVEGFNCYFPLQSYGFQPTNGVGYQPYRVVVLSFELLHAPATVCGPKGSPGSGSGSGYIPEAPRDGQAYVRKDGEWVLLSTFLGSGSGSEQYIKWPWYIWLGFIAGLIAIVMVTIMLCCMTSCCSCLKGCCSCGSCC

SEQ ID NO: 41 - RNA, 1406 nt, synthetic construct
  source 1..1406: mol_type = other RNA
agaataaactagtattcttctggtccccacagactcagagagaacccgccaccatggattggatttggagaatcctgttcctcgtgggagccgctacaggagcccactcccagatgcaggtgagatttccaaatattacaaatctgtgtccatttggagaagtgtttaatgcaacaagatttgcatctgtgtatgcatggaatagaaaaagaatttctaattgtgtggctgattattctgtgctgtataatagtgcttctttttccacatttaaatgttatggagtgtctccaacaaaattaaatgatttatgttttacaaatgtgtatgctgattcttttgtgatcagaggtgatgaagtgagacagattgcccccggacagacaggaaaaattgctgattacaattacaaactgcctgatgattttacaggatgtgtgattgcttggaattctaataatttagattctaaagtgggaggaaattacaattatctgtacagactgtttagaaaatcaaatctgaaaccttttgaaagagatatttcaacagaaatttatcaggctggatcaacaccttgtaatggagtggaaggatttaattgttattttccattacagagctatggatttcagccaaccaatggtgtgggatatcagccatatagagtggtggtgctgtcttttgaactgctgcatgcacctgcaacagtgtgtggacctaaaggctcccccggctccggctccggatctggttatattcctgaagctccaagagatgggcaagcttacgttcgtaaagatggcgaatgggtattactttctacctttttaggaagcggcagcggatctgaacagtacattaaatggccttggtacatttggcttggatttattgcaggattaattgcaattgtgatggtgacaattatgttatgttgtatgacatcatgttgttcttgtttaaaaggatgttgttcttgtggaagctgttgttgatgactcgagctggtactgcatgcacgcaatgctagctgcccctttcccgtcctgggtaccccgagtctcccccgacctcgggtcccaggtatgctcccacctccacctgccccactcaccacctctgctagttccagacacctcccaagcacgcagcaatgcagctcaaaacgcttagcctagccacacccccacgggaaacagcagtgattaacctttagcaataaacgaaagtttaactaagctatactaaccccagggttggtcaatttcgtgccagccacaccctggagctagcaaaaaaaaaaaaaaaaaaaaaaaaaaaaaagcatatgactaaaaaaaaaaaaaaaaaaaaaaaaaaaaaaaaaaaaaaaaaaaaaaaaaaaaaaaaaaaaaaaaaaaaaa